European Patent Application EP 4 223 874 A2, published August 9, 2023. Title: HUMAN ANTI-IL-33 NEUTRALIZING MONOCLONAL ANTIBODY. Applicant: Mitsubishi Tanabe Pharma Corporation. The sequence listing filed with the application follows.

SEQUENCE LISTING (427 sequences)

SEQ ID NO: 1 - protein, 14 aa, synthetic construct
  REGION 1..14: note = LCDR1-1
TGSSSNIGAVYDVH

SEQ ID NO: 2 - protein, 14 aa, synthetic construct
  REGION 1..14: note = LCDR1-2
TGSSSNIGAVYNVH

SEQ ID NO: 3 - protein, 13 aa, synthetic construct
  REGION 1..13: note = LCDR1-3
SGSSSNIGNNAVS

SEQ ID NO: 4 - protein, 13 aa, synthetic construct
  REGION 1..13: note = LCDR1-4
SGSSSNIGRNAVN

SEQ ID NO: 5 - protein, 13 aa, synthetic construct
  REGION 1..13: note = LCDR1-5
SGSCSNIGRNAVN

SEQ ID NO: 6 - protein, 13 aa, synthetic construct
  REGION 1..13: note = LCDR1-6
SGSSSNIGNNAVN

SEQ ID NO: 7 - protein, 13 aa, synthetic construct
  REGION 1..13: note = LCDR1-7
SGSSSNIGSNAVS

SEQ ID NO: 8 - protein, 13 aa, synthetic construct
  REGION 1..13: note = LCDR1-8
SGSSSNIGRNAVS

SEQ ID NO: 9 - protein, 13 aa, synthetic construct
  REGION 1..13: note = LCDR1-9
SGSSSNIGHNAVS

SEQ ID NO: 10 - protein, 13 aa, synthetic construct
  REGION 1..13: note = LCDR1-10
SGSSSNIGHNAVW

SEQ ID NO: 11 - protein, 7 aa, synthetic construct
  REGION 1..7: note = LCDR2-1
RNNQRPS

SEQ ID NO: 12 - protein, 7 aa, synthetic construct
  REGION 1..7: note = LCDR2-2
ASNMRVI

SEQ ID NO: 13 - protein, 7 aa, synthetic construct
  REGION 1..7: note = LCDR2-3
ASNMRVL

SEQ ID NO: 14 - protein, 7 aa, synthetic construct
  REGION 1..7: note = LCDR2-4
ASNMRGS

SEQ ID NO: 15 - protein, 7 aa, synthetic construct
  REGION 1..7: note = LCDR2-5
ASNMRVS

SEQ ID NO: 16 - protein, 7 aa, synthetic construct
  REGION 1..7: note = LCDR2-6
ASNMRGL

SEQ ID NO: 17 - protein, 7 aa, synthetic construct
  REGION 1..7: note = LCDR2-7
ASNMRRS

SEQ ID NO: 18 - protein, 7 aa, synthetic construct
  REGION 1..7: note = LCDR2-8
ASNMRRP

SEQ ID NO: 19 - protein, 7 aa, synthetic construct
  REGION 1..7: note = LCDR2-9
ASNMRRM

SEQ ID NO: 20 - protein, 7 aa, synthetic construct
  REGION 1..7: note = LCDR2-10
ASNMRRL

SEQ ID NO: 21 - protein, 7 aa, synthetic construct
  REGION 1..7: note = LCDR2-11
ASNMRGM

SEQ ID NO: 22 - protein, 9 aa, synthetic construct
  REGION 1..9: note = LCDR3-1
QTYDSSRWV

SEQ ID NO: 23 - protein, 9 aa, synthetic construct
  REGION 1..9: note = LCDR3-2
QSYDSSRWV

SEQ ID NO: 24 - protein, 9 aa, synthetic construct
  REGION 1..9: note = LCDR3-3
QSYDSRRWV

SEQ ID NO: 25 - protein, 11 aa, synthetic construct
  REGION 1..11: note = LCDR3-4
GAWDDSQKALV

SEQ ID NO: 26 - protein, 11 aa, synthetic construct
  REGION 1..11: note = LCDR3-5
AAWDDSQKAWV

SEQ ID NO: 27 - protein, 11 aa, synthetic construct
  REGION 1..11: note = LCDR3-6
WAWDDSQKAVV

SEQ ID NO: 28 - protein, 11 aa, synthetic construct
  REGION 1..11: note = LCDR3-7
EAWDDSQKGVV

SEQ ID NO: 29 - protein, 11 aa, synthetic construct
  REGION 1..11: note = LCDR3-8
GAWDDSQKRYV

SEQ ID NO: 30 - protein, 11 aa, synthetic construct
  REGION 1..11: note = LCDR3-9
AAWDDSQKGQV

SEQ ID NO: 31 - protein, 11 aa, synthetic construct
  REGION 1..11: note = LCDR3-10
AAWDDSQKVVV

SEQ ID NO: 32 - protein, 11 aa, synthetic construct
  REGION 1..11: note = LCDR3-11
WAWDDSQKVGV

SEQ ID NO: 33 - protein, 11 aa, synthetic construct
  REGION 1..11: note = LCDR3-12
GAWDDSQKVFV

SEQ ID NO: 34 - protein, 11 aa, synthetic construct
  REGION 1..11: note = LCDR3-13
SAWDDSQKVVV

SEQ ID NO: 35 - protein, 11 aa, synthetic construct
  REGION 1..11: note = LCDR3-14
EAWDDSQKAVV

SEQ ID NO: 36 - protein, 11 aa, synthetic construct
  REGION 1..11: note = LCDR3-15
AAWDDSQKAFV

SEQ ID NO: 37 - protein, 11 aa, synthetic construct
  REGION 1..11: note = LCDR3-16
AAWDDSQKVFV

SEQ ID NO: 38 - protein, 11 aa, synthetic construct
  REGION 1..11: note = LCDR3-17
GAWDDSQKAFV

SEQ ID NO: 39 - protein, 11 aa, synthetic construct
  REGION 1..11: note = LCDR3-18
GAWDDSQKVVV

SEQ ID NO: 40 - protein, 11 aa, synthetic construct
  REGION 1..11: note = LCDR3-19
AAWDDSQKAVV

SEQ ID NO: 41 - protein, 11 aa, synthetic construct
  REGION 1..11: note = LCDR3-20
SAWDDSQKAGV

SEQ ID NO: 42 - protein, 11 aa, synthetic construct
  REGION 1..11: note = LCDR3-21
AAWDDSQKALV

SEQ ID NO: 43 - protein, 5 aa, synthetic construct
  REGION 1..5: note = HCDR1-1
DYYMN

SEQ ID NO: 44 - protein, 5 aa, synthetic construct
  REGION 1..5: note = HCDR1-2
DYYMD

SEQ ID NO: 45 - protein, 5 aa, synthetic construct
  REGION 1..5: note = HCDR1-3
VYYMN

SEQ ID NO: 46 - protein, 5 aa, synthetic construct
  REGION 1..5: note = HCDR1-4
DYYVN

SEQ ID NO: 47 - protein, 5 aa, synthetic construct
  REGION 1..5: note = HCDR1-5
NYYMH

SEQ ID NO: 48 - protein, 5 aa, synthetic construct
  REGION 1..5: note = HCDR1-6
HYYMH

SEQ ID NO: 49 - protein, 5 aa, synthetic construct
  REGION 1..5: note = HCDR1-7
RYYMH

SEQ ID NO: 50 - protein, 5 aa, synthetic construct
  REGION 1..5: note = HCDR1-8
SYYMH

SEQ ID NO: 51 - protein, 17 aa, synthetic construct
  REGION 1..17: note = HCDR2-1
SISRYSSYIYYADSVKG

SEQ ID NO: 52 - protein, 17 aa, synthetic construct
  REGION 1..17: note = HCDR2-2
SISRYSGYVYYADSVKG

SEQ ID NO: 53 - protein, 17 aa, synthetic construct
  REGION 1..17: note = HCDR2-3
SISRASSYVYYADSVKG

SEQ ID NO: 54 - protein, 17 aa, synthetic construct
  REGION 1..17: note = HCDR2-4
SISRYSGYIYYADSVKG

SEQ ID NO: 55 - protein, 17 aa, synthetic construct
  REGION 1..17: note = HCDR2-5
SISARSRYHYYADSVKG

SEQ ID NO: 56 - protein, 17 aa, synthetic construct
  REGION 1..17: note = HCDR2-6
SISARSSYIYYADSVKG

SEQ ID NO: 57 - protein, 17 aa, synthetic construct
  REGION 1..17: note = HCDR2-7
SISALSSYIYYADSVRG

SEQ ID NO: 58 - protein, 17 aa, synthetic construct
  REGION 1..17: note = HCDR2-8
SISAQSSHIYYADSVEG

SEQ ID NO: 59 - protein, 17 aa, synthetic construct
  REGION 1..17: note = HCDR2-9
SISARSSYLYYADSVKG

SEQ ID NO: 60 - protein, 17 aa, synthetic construct
  REGION 1..17: note = HCDR2-10
SISARSSYRYYADSVKG

SEQ ID NO: 61 - protein, 17 aa, synthetic construct
  REGION 1..17: note = HCDR2-11
SISARSSYIYYAGSVKG

SEQ ID NO: 62 - protein, 17 aa, synthetic construct
  REGION 1..17: note = HCDR2-12
SISSRSSHQYYAGSVKG

SEQ ID NO: 63 - protein, 17 aa, synthetic construct
  REGION 1..17: note = HCDR2-13
SISALSSYRYYADSVKG

SEQ ID NO: 64 - protein, 17 aa, synthetic construct
  REGION 1..17: note = HCDR2-14
SISSSSSYIYYADSVKG

SEQ ID NO: 65 - protein, 7 aa, synthetic construct
  REGION 1..7: note = HCDR3-1
DIGGMDV

SEQ ID NO: 66 - protein, 10 aa, synthetic construct
  REGION 1..10: note = HCDR3-2
LATRHNAFDI

SEQ ID NO: 67 - protein, 10 aa, synthetic construct
  REGION 1..10: note = HCDR3-3
LATRNNAFDI

SEQ ID NO: 68 - protein, 10 aa, synthetic construct
  REGION 1..10: note = HCDR3-4
LATRRDAFDI

SEQ ID NO: 69 - protein, 10 aa, synthetic construct
  REGION 1..10: note = HCDR3-5
LATRQNAFDI

SEQ ID NO: 70 - protein, 10 aa, synthetic construct
  REGION 1..10: note = HCDR3-6
LATRHVAFDI

SEQ ID NO: 71 - protein, 10 aa, synthetic construct
  REGION 1..10: note = HCDR3-7
LATRHGAFDI

SEQ ID NO: 72 - protein, 10 aa, synthetic construct
  REGION 1..10: note = HCDR3-8
LATRHLAFDI

SEQ ID NO: 73 - protein, 10 aa, synthetic construct
  REGION 1..10: note = HCDR3-9
LATRHSAFDI

SEQ ID NO: 74 - protein, 10 aa, synthetic construct
  REGION 1..10: note = HCDR3-10
LGTRRVAFDI

SEQ ID NO: 75 - protein, 10 aa, synthetic construct
  REGION 1..10: note = HCDR3-11
LGLRHDAFDI

SEQ ID NO: 76 - protein, 10 aa, synthetic construct
  REGION 1..10: note = HCDR3-12
LATRRIAFDI

SEQ ID NO: 77 - protein, 10 aa, synthetic construct
  REGION 1..10: note = HCDR3-13
LATRRVAFDI

SEQ ID NO: 78 - protein, 10 aa, synthetic construct
  REGION 1..10: note = HCDR3-14
LGTRHDAFDI

SEQ ID NO: 79 - protein, 109 aa, synthetic construct
  REGION 1..109: note = VL-1
QSVLTQPPSASGTPGQRVTISCTGSSSNIGAVYDVHWYQQLPGTAPKLLIYRNNQRPSGVPDRFSGSKSGTSASLAISGLRSEDEADYYCQTYDSSRWVFGGGTKLTVL

SEQ ID NO: 80 - protein, 109 aa, synthetic construct
  REGION 1..109: note = VL-2
QSVLTQPPSASGTPGQRVTISCTGSSSNIGAVYDVHWYQQLPGTAPKLLIYRNNQRPSGVPDRFSGSKSGTSASLAISGLRSEDEADYYCQSYDSSRWVFGGGTKLTVL

SEQ ID NO: 81 - protein, 109 aa, synthetic construct
  REGION 1..109: note = VL-3
QSVLTQPPSASGTPGQRVTISCTGSSSNIGAVYNVHWYQQLPGTAPKLLIYRNNQRPSGVPDRFSGSKSGTSASLAISGLRSEDEADYYCQSYDSSRWVFGGGTKLTVL

SEQ ID NO: 82 - protein, 109 aa, synthetic construct
  REGION 1..109: note = VL-4
QSVLTQPPSASGTPGQRVTISCTGSSSNIGAVYNVHWYQQLPGTAPKLLIYRNNQRPSGVPDRFSGSKSGTSASLAISGLRSEDEADYYCQSYDSRRWVFGGGTKLTVL

SEQ ID NO: 83 - protein, 110 aa, synthetic construct
  REGION 1..110: note = VL-5
QSVLTQPPSASGTPGQRVTISCSGSSSNIGNNAVSWYQQLPGTAPKLLIYASNMRVIGVPDRFSGSKSGTSASLAISGLRSEDEADYYCGAWDDSQKALVFGGGTKLTVL

SEQ ID NO: 84 - protein, 110 aa, synthetic construct
  REGION 1..110: note = VL-6
QSVLTQPPSASGTPGQRVTISCSGSSSNIGRNAVNWYQQLPGTAPKLLIYASNMRVIGVPDRFSGSKSGTSASLAISGLRSEDEADYYCAAWDDSQKAWVFGGGTKLTVL

SEQ ID NO: 85 - protein, 110 aa, synthetic construct
  REGION 1..110: note = VL-7
QSVLTQPPSASGTPGQRVTISCSGSSSNIGRNAVNWYQQLPGTAPKLLIYASNMRVLGVPDRFSGSKSGTSASLAISGLRSEDEADYYCWAWDDSQKAVVFGGGTKLTVL

SEQ ID NO: 86 - protein, 110 aa, synthetic construct
  REGION 1..110: note = VL-8
QSVLTQPPSASGTPGQRVTISCSGSCSNIGRNAVNWYQQLPGTAPKLLIYASNMRVIGVPDRFSGSKSGTSASLAISGLRSEDEADYYCEAWDDSQKGVVFGGGTKLTVL

SEQ ID NO: 87 - protein, 110 aa, synthetic construct
  REGION 1..110: note = VL-9
QSVLTQPPSASGTPGQRVTISCSGSSSNIGRNAVNWYQQLPGTAPKLLIYASNMRVIGVPDRFSGSKSGTSASLAISGLRSEDEADYYCGAWDDSQKRYVFGGGTKLTVL

SEQ ID NO: 88 - protein, 110 aa, synthetic construct
  REGION 1..110: note = VL-10
QSVLTQPPSASGTPGQRVTISCSGSSSNIGNNAVNWYQQLPGTAPKLLIYASNMRGSGVPDRFSGSKSGTSASLAISGLRSEDEADYYCAAWDDSQKGQVFGGGTKLTVL

SEQ ID NO: 89 - protein, 110 aa, synthetic construct
  REGION 1..110: note = VL-11
QSVLTQPPSASGTPGQRVTISCSGSSSNIGSNAVSWYQQLPGTAPKLLIYASNMRGSGVPDRFSGSKSGTSASLAISGLRSEDEADYYCAAWDDSQKVVVFGGGTKLTVL

SEQ ID NO: 90 - protein, 110 aa, synthetic construct
  REGION 1..110: note = VL-12
QSVLTQPPSASGTPGQRVTISCSGSSSNIGRNAVNWYQQLPGTAPKLLIYASNMRVSGVPDRFSGSKSGTSASLAISGLRSEDEADYYCWAWDDSQKVGVFGGGTKLTVL

SEQ ID NO: 91 - protein, 110 aa, synthetic construct
  REGION 1..110: note = VL-13
QSVLTQPPSASGTPGQRVTISCSGSSSNIGNNAVNWYQQLPGTAPKLLIYASNMRGLGVPDRFSGSKSGTSASLAISGLRSEDEADYYCGAWDDSQKVFVFGGGTKLTVL

SEQ ID NO: 92 - protein, 110 aa, synthetic construct
  REGION 1..110: note = VL-14
QSVLTQPPSASGTPGQRVTISCSGSSSNIGRNAVNWYQQLPGTAPKLLIYASNMRRSGVPDRFSGSKSGTSASLAISGLRSEDEADYYCSAWDDSQKVVVFGGGTKLTVL

SEQ ID NO: 93 - protein, 110 aa, synthetic construct
  REGION 1..110: note = VL-15
QSVLTQPPSASGTPGQRVTISCSGSSSNIGNNAVNWYQQLPGTAPKLLIYASNMRRPGVPDRFSGSKSGTSASLAISGLRSEDEADYYCEAWDDSQKAVVFGGGTKLTVL

SEQ ID NO: 94 - protein, 110 aa, synthetic construct
  REGION 1..110: note = VL-16
QSVLTQPPSASGTPGQRVTISCSGSSSNIGNNAVNWYQQLPGTAPKLLIYASNMRRMGVPDRFSGSKSGTSASLAISGLRSEDEADYYCAAWDDSQKAFVFGGGTKLTVL

SEQ ID NO: 95 - protein, 110 aa, synthetic construct
  REGION 1..110: note = VL-17
QSVLTQPPSASGTPGQRVTISCSGSSSNIGNNAVNWYQQLPGTAPKLLIYASNMRRLGVPDRFSGSKSGTSASLAISGLRSEDEADYYCAAWDDSQKAWVFGGGTKLTVL

SEQ ID NO: 96 - protein, 110 aa, synthetic construct
  REGION 1..110: note = VL-18
QSVLTQPPSASGTPGQRVTISCSGSSSNIGNNAVNWYQQLPGTAPKLLIYASNMRRPGVPDRFSGSKSGTSASLAISGLRSEDEADYYCAAWDDSQKVFVFGGGTKLTVL

SEQ ID NO: 97 - protein, 110 aa, synthetic construct
  REGION 1..110: note = VL-19
QSVLTQPPSASGTPGQRVTISCSGSSSNIGNNAVNWYQQLPGTAPKLLIYASNMRRLGVPDRFSGSKSGTSASLAISGLRSEDEADYYCGAWDDSQKAFVFGGGTKLTVL

SEQ ID NO: 98 - protein, 110 aa, synthetic construct
  REGION 1..110: note = VL-20
QSVLTQPPSASGTPGQRVTISCSGSSSNIGRNAVSWYQQLPGTAPKLLIYASNMRRLGVPDRFSGSKSGTSASLAISGLRSEDEADYYCWAWDDSQKAVVFGGGTKLTVL

SEQ ID NO: 99 - protein, 110 aa, synthetic construct
  REGION 1..110: note = VL-21
QSVLTQPPSASGTPGQRVTISCSGSSSNIGHNAVSWYQQLPGTAPKLLIYASNMRRLGVPDRFSGSKSGTSASLAISGLRSEDEADYYCGAWDDSQKVVVFGGGTKLTVL

SEQ ID NO: 100 - protein, 110 aa, synthetic construct
  REGION 1..110: note = VL-22
QSVLTQPPSASGTPGQRVTISCSGSSSNIGRNAVNWYQQLPGTAPKLLIYASNMRGMGVPDRFSGSKSGTSASLAISGLRSEDEADYYCSAWDDSQKVVVFGGGTKLTVL

SEQ ID NO: 101 - protein, 110 aa, synthetic construct
  REGION 1..110: note = VL-23
QSVLTQPPSASGTPGQRVTISCSGSSSNIGHNAVWWYQQLPGTAPKLLIYASNMRRMGVPDRFSGSKSGTSASLAISGLRSEDEADYYCAAWDDSQKAVVFGGGTKLTVL

SEQ ID NO: 102 - protein, 110 aa, synthetic construct
  REGION 1..110: note = VL-24
QSVLTQPPSASGTPGQRVTISCSGSSSNIGRNAVNWYQQLPGTAPKLLIYASNMRRPGVPDRFSGSKSGTSASLAISGLRSEDEADYYCSAWDDSQKAGVFGGGTKLTVL

SEQ ID NO: 103 - protein, 110 aa, synthetic construct
  REGION 1..110: note = VL-25
QSVLTQPPSASGTPGQRVTISCSGSSSNIGNNAVNWYQQLPGTAPKLLIYASNMRRLGVPDRFSGSKSGTSASLAISGLRSEDEADYYCAAWDDSQKALVFGGGTKLTVL

SEQ ID NO: 104 - protein, 110 aa, synthetic construct
  REGION 1..110: note = VL-26
QSVLTQPPSASGTPGQRVTISCSGSSSNIGNNAVNWYQQLPGTAPKLLIYASNMRRLGVPDRFSGSKSGTSASLAISGLRSEDEADYYCAAWDDSQKAVVFGGGTKLTVL

SEQ ID NO: 105 - protein, 116 aa, synthetic construct
  REGION 1..116: note = VH-1
EVQLLESGGGLVQPGGSLRLSCAASGFTFSDYYMNWVRQAPGKGLEWVSSISRYSSYIYYADSVKGRFTISRDNSKNTLYLQMNSLRAEDTAVYYCARDIGGMDVWGQGTLVTVSS

SEQ ID NO: 106 - protein, 116 aa, synthetic construct
  REGION 1..116: note = VH-2
EVQLLESGGGLVQPGGSLRLSCAASGFTFSDYYMNWVRQAPGKGLEWVSSISRYSGYVYYADSVKGRFTISRDNSKNTLYLQMNSLRAEDTAVYYCARDIGGMDVWGQGTLVTVSS

SEQ ID NO: 107 - protein, 116 aa, synthetic construct
  REGION 1..116: note = VH-3
EVQLLESGGGLVQPGGSLRLSCAASGFTFSDYYMDWVRQAPGKGLEWVSSISRYSGYVYYADSVKGRFTISRDNSKNTLYLQMNSLRAEDTAVYYCARDIGGMDVWGQGTLVTVSS

SEQ ID NO: 108 - protein, 116 aa, synthetic construct
  REGION 1..116: note = VH-4
EVQLLESGGGLVQPGGSLRLSCAASGFTFSDYYMDWVRQAPGKGLEWVSSISRASSYVYYADSVKGRFTISRDNSKNTLYLQMNSLRAEDTAVYYCARDIGGMDVWGQGTLVTVSS

SEQ ID NO: 109 - protein, 116 aa, synthetic construct
  REGION 1..116: note = VH-5
EVQLLESGGGLVQPGGSLRLSCAASGFTFSDYYMNWVRQAPGKGLEWVSSISRYSGYIYYADSVKGRFTISRDNSKNTLYLQMNSLRAEDTAVYYCARDIGGMDVWGQGTLVTVSS

SEQ ID NO: 110 - protein, 116 aa, synthetic construct
  REGION 1..116: note = VH-6
EVQLLESGGGLVQPGGSLRLSCAASGFTFSVYYMNWVRQAPGKGLEWVSSISRYSGYVYYADSVKGRFTISRDNSKNTLYLQMNSLRAEDTAVYYCARDIGGMDVWGQGTLVTVSS

SEQ ID NO: 111 - protein, 116 aa, synthetic construct
  REGION 1..116: note = VH-7
EVQLLESGGGLVQPGGSLRLSCAASGFTFSDYYVNWVRQAPGKGLEWVSSISRYSGYVYYADSVKGRFTISRDNSKNTLYLQMNSLRAEDTAVYYCARDIGGMDVWGQGTLVTVSS

SEQ ID NO: 112 - protein, 119 aa, synthetic construct
  REGION 1..119: note = VH-8
EVQLLESGGGLVQPGGSLRLSCAASGFTFSNYYMHWVRQAPGKGLEWVSSISARSRYHYYADSVKGRFTISRDNSKNTLYLQMNSLRAEDTAVYYCARLATRHNAFDIWGQGTLVTVSS

SEQ ID NO: 113 - protein, 119 aa, synthetic construct
  REGION 1..119: note = VH-9
EVQLLESGGGLVQPGGSLRLSCAASGFTFSNYYMHWVRQAPGKGLEWVSSISARSSYIYYADSVKGRFTISRDNSKNTLYLQMNSLRAEDTAVYYCARLATRNNAFDIWGQGTLVTVSS

SEQ ID NO: 114 - protein, 119 aa, synthetic construct
  REGION 1..119: note = VH-10
EVQLLESGGGLVQPGGSLRLSCAASGFTFSHYYMHWVRQAPGKGLEWVSSISALSSYIYYADSVRGRFTISRDNSKNTLYLQMNSLRAEDTAVYYCARLATRRDAFDIWGQGTLVTVSS

SEQ ID NO: 115 - protein, 119 aa, synthetic construct
  REGION 1..119: note = VH-11
EVQLLESGGGLVQPGGSLRLSCAASGFTFSRYYMHWVRQAPGKGLEWVSSISAQSSHIYYADSVEGRFTISRDNSKNTLYLQMNSLRAEDTAVYYCARLATRQNAFDIWGQGTLVTVSS

SEQ ID NO: 116 - protein, 119 aa, synthetic construct
  REGION 1..119: note = VH-12
EVQLLESGGGLVQPGGSLRLSCAASGFTFSNYYMHWVRQAPGKGLEWVSSISARSSYLYYADSVKGRFTISRDNSKNTLYLQMNSLRAEDTAVYYCARLATRHVAFDIWGQGTLVTVSS

SEQ ID NO: 117 - protein, 119 aa, synthetic construct
  REGION 1..119: note = VH-13
EVQLLESGGGLVQPGGSLRLSCAASGFTFSNYYMHWVRQAPGKGLEWVSSISARSSYIYYADSVKGRFTISRDNSKNTLYLQMNSLRAEDTAVYYCARLATRHGAFDIWGQGTLVTVSS

SEQ ID NO: 118 - protein, 119 aa, synthetic construct
  REGION 1..119: note = VH-14
EVQLLESGGGLVQPGGSLRLSCAASGFTFSNYYMHWVRQAPGKGLEWVSSISARSSYIYYADSVKGRFTISRDNSKNTLYLQMNSLRAEDTAVYYCARLATRHNAFDIWGQGTLVTVSS

SEQ ID NO: 119 - protein, 119 aa, synthetic construct
  REGION 1..119: note = VH-15
EVQLLESGGGLVQPGGSLRLSCAASGFTFSNYYMHWVRQAPGKGLEWVSSISARSSYRYYADSVKGRFTISRDNSKNTLYLQMNSLRAEDTAVYYCARLATRHLAFDIWGQGTLVTVSS

SEQ ID NO: 120 - protein, 119 aa, synthetic construct
  REGION 1..119: note = VH-16
EVQLLESGGGLVQPGGSLRLSCAASGFTFSNYYMHWVRQAPGKGLEWVSSISARSSYIYYADSVKGRFTISRDNSKNTLYLQMNSLRAEDTAVYYCARLATRHSAFDIWGQGTLVTVSS

SEQ ID NO: 121 - protein, 119 aa, synthetic construct
  REGION 1..119: note = VH-17
EVQLLESGGGLVQPGGSLRLSCAASGFTFSRYYMHWVRQAPGKGLEWVSSISARSSYIYYADSVKGRFTISRDNSKNTLYLQMNSLRAEDTAVYYCARLATRRDAFDIWGQGTLVTVSS

SEQ ID NO: 122 - protein, 119 aa, synthetic construct
  REGION 1..119: note = VH-18
EVQLLESGGGLVQPGGSLRLSCAASGFTFSNYYMHWVRQAPGKGLEWVSSISARSSYRYYADSVKGRFTISRDNSKNTLYLQMNSLRAEDTAVYYCARLATRHSAFDIWGQGTLVTVSS

SEQ ID NO: 123 - protein, 119 aa, synthetic construct
  REGION 1..119: note = VH-19
EVQLLESGGGLVQPGGSLRLSCAASGFTFSNYYMHWVRQAPGKGLEWVSSISARSSYIYYAGSVKGRFTISRDNSKNTLYLQMNSLRAEDTAVYYCARLGTRRVAFDIWGQGTLVTVSS

SEQ ID NO: 124 - protein, 119 aa, synthetic construct
  REGION 1..119: note = VH-20
EVQLLESGGGLVQPGGSLRLSCAASGFTFSNYYMHWVRQAPGKGLEWVSSISSRSSHQYYAGSVKGRFTISRDNSKNTLYLQMNSLRAEDTAVYYCARLGLRHDAFDIWGQGTLVTVSS

SEQ ID NO: 125 - protein, 119 aa, synthetic construct
  REGION 1..119: note = VH-21
EVQLLESGGGLVQPGGSLRLSCAASGFTFSSYYMHWVRQAPGKGLEWVSSISARSSYIYYADSVKGRFTISRDNSKNTLYLQMNSLRAEDTAVYYCARLATRRIAFDIWGQGTLVTVSS

SEQ ID NO: 126 - protein, 119 aa, synthetic construct
  REGION 1..119: note = VH-22
EVQLLESGGGLVQPGGSLRLSCAASGFTFSNYYMHWVRQAPGKGLEWVSSISALSSYRYYADSVKGRFTISRDNSKNTLYLQMNSLRAEDTAVYYCARLATRRVAFDIWGQGTLVTVSS

SEQ ID NO: 127 - protein, 116 aa, synthetic construct
  REGION 1..116: note = VH-23
EVQLLESGGGLVQPGGSLRLSCAASGFTFSDYYMNWVRQAPGKGLEWVSSISSSSSYIYYADSVKGRFTISRDNSKNTLYLQMNSLRAEDTAVYYCARDIGGMDVWGQGTLVTVSS

SEQ ID NO: 128 - protein, 119 aa, synthetic construct
  REGION 1..119: note = VH-24
EVQLLESGGGLVQPGGSLRLSCAASGFTFSNYYMHWVRQAPGKGLEWVSSISSSSSYIYYADSVKGRFTISRDNSKNTLYLQMNSLRAEDTAVYYCARLGTRHDAFDIWGQGTLVTVSS

SEQ ID NO: 129 - DNA, 42 bp, synthetic construct
  misc_feature 1..42: note = N-LCDR1-1
  source 1..42: mol_type = other DNA
actgggagcagctccaacatcggggcagtttatgatgtacac

SEQ ID NO: 130 - DNA, 42 bp, synthetic construct
  misc_feature 1..42: note = N-LCDR1-2
  source 1..42: mol_type = other DNA
actgggagcagctccaacatcggggcagtttataatgtacac

SEQ ID NO: 131 - DNA, 39 bp, synthetic construct
  misc_feature 1..39: note = N-LCDR1-3
  source 1..39: mol_type = other DNA
tctggaagcagctccaacatcggaaataatgctgtaagc

SEQ ID NO: 132 - DNA, 39 bp, synthetic construct
  misc_feature 1..39: note = N-LCDR1-4
  source 1..39: mol_type = other DNA
tctggaagcagctccaacatcggacgtaatgctgtaaac

SEQ ID NO: 133 - DNA, 39 bp, synthetic construct
  misc_feature 1..39: note = N-LCDR1-5
  source 1..39: mol_type = other DNA
tctggaagctgctccaacatcggacgtaatgctgtaaac

SEQ ID NO: 134 - DNA, 39 bp, synthetic construct
  misc_feature 1..39: note = N-LCDR1-6
  source 1..39: mol_type = other DNA
tctggaagcagctccaacatcggaaataatgctgtaaac

SEQ ID NO: 135 - DNA, 39 bp, synthetic construct
  misc_feature 1..39: note = N-LCDR1-7
  source 1..39: mol_type = other DNA
tctggaagcagctccaacatcggaagtaatgctgtaagc

SEQ ID NO: 136 - DNA, 39 bp, synthetic construct
  misc_feature 1..39: note = N-LCDR1-8
  source 1..39: mol_type = other DNA
tctggaagcagctccaacatcggacgcaatgctgtaagc

SEQ ID NO: 137 - DNA, 39 bp, synthetic construct
  misc_feature 1..39: note = N-LCDR1-9
  source 1..39: mol_type = other DNA
tctggaagcagctccaacatcggacacaatgctgtaagc

SEQ ID NO: 138 - DNA, 39 bp, synthetic construct
  misc_feature 1..39: note = N-LCDR1-10
  source 1..39: mol_type = other DNA
tctggaagcagctccaacatcggacgcaatgctgtaaac

SEQ ID NO: 139 - DNA, 39 bp, synthetic construct
  misc_feature 1..39: note = N-LCDR1-11
  source 1..39: mol_type = other DNA
tctggaagcagctccaacatcggacacaatgctgtatgg

SEQ ID NO: 140 - DNA, 21 bp, synthetic construct
  misc_feature 1..21: note = N-LCDR1-12
  source 1..21: mol_type = other DNA
aggaataatcagcggccctca

SEQ ID NO: 141 - DNA, 21 bp, synthetic construct
  misc_feature 1..21: note = N-LCDR2-1
  source 1..21: mol_type = other DNA
gccagtaacatgagagtcatt

SEQ ID NO: 142 - DNA, 21 bp, synthetic construct
  misc_feature 1..21: note = N-LCDR2-2
  source 1..21: mol_type = other DNA
gccagtaacatgagagtctta

SEQ ID NO: 143 - DNA, 21 bp, synthetic construct
  misc_feature 1..21: note = N-LCDR2-3
  source 1..21: mol_type = other DNA
gccagtaacatgagagtcata

SEQ ID NO: 144 - DNA, 21 bp, synthetic construct
  misc_feature 1..21: note = N-LCDR2-4
  source 1..21: mol_type = other DNA
gccagtaacatgagaggctct

SEQ ID NO: 145 - DNA, 21 bp, synthetic construct
  misc_feature 1..21: note = N-LCDR2-5
  source 1..21: mol_type = other DNA
gccagtaacatgagagtctct

SEQ ID NO: 146 - DNA, 21 bp, synthetic construct
  misc_feature 1..21: note = N-LCDR2-6
  source 1..21: mol_type = other DNA
gccagtaacatgagaggctta

SEQ ID NO: 147 - DNA, 21 bp, synthetic construct
  misc_feature 1..21: note = N-LCDR2-7
  source 1..21: mol_type = other DNA
gccagtaacatgagacgctct

SEQ ID NO: 148 - DNA, 21 bp, synthetic construct
  misc_feature 1..21: note = N-LCDR2-8
  source 1..21: mol_type = other DNA
gccagtaacatgagacgcccg

SEQ ID NO: 149 - DNA, 21 bp, synthetic construct
  misc_feature 1..21: note = N-LCDR2-9
  source 1..21: mol_type = other DNA
gccagtaacatgagacgcatg

SEQ ID NO: 150 - DNA, 21 bp, synthetic construct
  misc_feature 1..21: note = N-LCDR2-10
  source 1..21: mol_type = other DNA
gccagtaacatgagacgcctg

SEQ ID NO: 151 - DNA, 21 bp, synthetic construct
  misc_feature 1..21: note = N-LCDR2-11
  source 1..21: mol_type = other DNA
gccagtaacatgagacgtctg

SEQ ID NO: 152 - DNA, 21 bp, synthetic construct
  misc_feature 1..21: note = N-LCDR2-12
  source 1..21: mol_type = other DNA
gccagtaacatgagaggtatg

SEQ ID NO: 153 - DNA, 21 bp, synthetic construct
  misc_feature 1..21: note = N-LCDR2-13
  source 1..21: mol_type = other DNA
gccagtaacatgagacgtatg

SEQ ID NO: 154 - DNA, 21 bp, synthetic construct
  misc_feature 1..21: note = N-LCDR2-14
  source 1..21: mol_type = other DNA
gccagtaacatgagacgtccg

SEQ ID NO: 155 - DNA, 21 bp, synthetic construct
  misc_feature 1..21: note = N-LCDR2-15
  source 1..21: mol_type = other DNA
gccagtaacatgagacgctta

SEQ ID NO: 156 - DNA, 27 bp, synthetic construct
  misc_feature 1..27: note = N-LCDR3-1
  source 1..27: mol_type = other DNA
cagacttatgacagcagccgttgggtg

SEQ ID NO: 157 - DNA, 27 bp, synthetic construct
  misc_feature 1..27: note = N-LCDR3-2
  source 1..27: mol_type = other DNA
cagtcctatgacagcagccgttgggtg

SEQ ID NO: 158 - DNA, 27 bp, synthetic construct
  misc_feature 1..27: note = N-LCDR3-3
  source 1..27: mol_type = other DNA
cagtcctatgacagccgccgttgggtg

SEQ ID NO: 159 - DNA, 33 bp, synthetic construct
  misc_feature 1..33: note = N-LCDR3-4
  source 1..33: mol_type = other DNA
ggagcatgggatgacagccagaaggctcttgtt

SEQ ID NO: 160 - DNA, 33 bp, synthetic construct
  misc_feature 1..33: note = N-LCDR3-5
  source 1..33: mol_type = other DNA
gcagcatgggatgacagccagaaggcttgggtt

SEQ ID NO: 161 - DNA, 33 bp, synthetic construct
  misc_feature 1..33: note = N-LCDR3-6
  source 1..33: mol_type = other DNA
tgggcatgggatgacagccagaaggctgtggtt

SEQ ID NO: 162 - DNA, 33 bp, synthetic construct
  misc_feature 1..33: note = N-LCDR3-7
  source 1..33: mol_type = other DNA
gaggcatgggatgacagccagaagggtgtggtt

SEQ ID NO: 163 - DNA, 33 bp, synthetic construct
  misc_feature 1..33: note = N-LCDR3-8
  source 1..33: mol_type = other DNA
ggagcatgggatgacagccagaagcgttatgtt

SEQ ID NO: 164 - DNA, 33 bp, synthetic construct
  misc_feature 1..33: note = N-LCDR3-9
  source 1..33: mol_type = other DNA
gcggcatgggatgacagccagaagggtcaggtt

SEQ ID NO: 165 - DNA, 33 bp, synthetic construct
  misc_feature 1..33: note = N-LCDR3-10
  source 1..33: mol_type = other DNA
gcagcatgggatgacagccagaaggttgtggtt

SEQ ID NO: 166 - DNA, 33 bp, synthetic construct
  misc_feature 1..33: note = N-LCDR3-11
  source 1..33: mol_type = other DNA
tgggcatgggatgacagccagaaggttggtgtt

SEQ ID NO: 167 - DNA, 33 bp, synthetic construct
  misc_feature 1..33: note = N-LCDR3-12
  source 1..33: mol_type = other DNA
ggggcatgggatgacagccagaaggtttttgtt

SEQ ID NO: 168 - DNA, 33 bp, synthetic construct
  misc_feature 1..33: note = N-LCDR3-13
  source 1..33: mol_type = other DNA
tcagcatgggatgacagccagaaggttgtggtt

SEQ ID NO: 169 - DNA, 33 bp, synthetic construct
  misc_feature 1..33: note = N-LCDR3-14
  source 1..33: mol_type = other DNA
gaggcatgggatgacagccagaaggctgttgtt

SEQ ID NO: 170 - DNA, 33 bp, synthetic construct
  misc_feature 1..33: note = N-LCDR3-15
  source 1..33: mol_type = other DNA
gcggcatgggatgacagccagaaggcttttgtt

SEQ ID NO: 171 - DNA, 33 bp, synthetic construct
  misc_feature 1..33: note = N-LCDR3-16
  source 1..33: mol_type = other DNA
gcggcatgggatgacagccagaaggcttgggtt

SEQ ID NO: 172 - DNA, 33 bp, synthetic construct
  misc_feature 1..33: note = N-LCDR3-17
  source 1..33: mol_type = other DNA
gcggcatgggatgacagccagaaggtttttgtt

SEQ ID NO: 173 - DNA, 33 bp, synthetic construct
  misc_feature 1..33: note = N-LCDR3-18
  source 1..33: mol_type = other DNA
ggggcatgggatgacagccagaaggcttttgtt

SEQ ID NO: 174 - DNA, 33 bp, synthetic construct
  misc_feature 1..33: note = N-LCDR3-19
  source 1..33: mol_type = other DNA
tgggcatgggatgacagccagaaggctgttgtt

SEQ ID NO: 175 - DNA, 33 bp, synthetic construct
  misc_feature 1..33: note = N-LCDR3-20
  source 1..33: mol_type = other DNA
ggggcatgggatgacagccagaaggttgtggtt

SEQ ID NO: 176 - DNA, 33 bp, synthetic construct
  misc_feature 1..33: note = N-LCDR3-21
  source 1..33: mol_type = other DNA
tcggcatgggatgacagccagaaggttgttgtt

SEQ ID NO: 177 - DNA, 33 bp, synthetic construct
  misc_feature 1..33: note = N-LCDR3-22
  source 1..33: mol_type = other DNA
gcggcatgggatgacagccagaaggctgttgtt

SEQ ID NO: 178 - DNA, 33 bp, synthetic construct
  misc_feature 1..33: note = N-LCDR3-23
  source 1..33: mol_type = other DNA
tcggcatgggatgacagccagaaggctggggtt

SEQ ID NO: 179 - DNA, 33 bp, synthetic construct
  misc_feature 1..33: note = N-LCDR3-24
  source 1..33: mol_type = other DNA
gcggcatgggatgacagccagaaggctttggtt

SEQ ID NO: 180 - DNA, 33 bp, synthetic construct
  misc_feature 1..33: note = N-LCDR3-25
  source 1..33: mol_type = other DNA
gcagcatgggatgacagccagaaggctgttgtt

SEQ ID NO: 181 - DNA, 15 bp, synthetic construct
  misc_feature 1..15: note = N-HCDR1-1
  source 1..15: mol_type = other DNA
gactactacatgaac

SEQ ID NO: 182 - DNA, 15 bp, synthetic construct
  misc_feature 1..15: note = N-HCDR1-2
  source 1..15: mol_type = other DNA
gactactacatggac

SEQ ID NO: 183 - DNA, 15 bp, synthetic construct
  misc_feature 1..15: note = N-HCDR1-3
  source 1..15: mol_type = other DNA
gtctactacatgaac

SEQ ID NO: 184 - DNA, 15 bp, synthetic construct
  misc_feature 1..15: note = N-HCDR1-4
  source 1..15: mol_type = other DNA
gactactacgtgaac

SEQ ID NO: 185 - DNA, 15 bp, synthetic construct
  misc_feature 1..15: note = N-HCDR1-5
  source 1..15: mol_type = other DNA
aattactacatgcac

SEQ ID NO: 186 - DNA, 15 bp, synthetic construct
  misc_feature 1..15: note = N-HCDR1-6
  source 1..15: mol_type = other DNA
cattactacatgcac

SEQ ID NO: 187 - DNA, 15 bp, synthetic construct
  misc_feature 1..15: note = N-HCDR1-7
  source 1..15: mol_type = other DNA
cgttactacatgcac

SEQ ID NO: 188 - DNA, 15 bp, synthetic construct
  misc_feature 1..15: note = N-HCDR1-8
  source 1..15: mol_type = other DNA
cgctactacatgcac

SEQ ID NO: 189 - DNA, 15 bp, synthetic construct
  misc_feature 1..15: note = N-HCDR1-9
  source 1..15: mol_type = other DNA
aactactacatgcac

SEQ ID NO: 190 - DNA, 15 bp, synthetic construct
  misc_feature 1..15: note = N-HCDR1-10
  source 1..15: mol_type = other DNA
agctactacatgcac

SEQ ID NO: 191 - DNA, 51 bp, synthetic construct
  misc_feature 1..51: note = N-HCDR2-1
  source 1..51: mol_type = other DNA
tccattagtcggtatagtagttacatatactacgcagactcagtgaagggc

SEQ ID NO: 192 - DNA, 51 bp, synthetic construct
  misc_feature 1..51: note = N-HCDR2-2
  source 1..51: mol_type = other DNA
tccattagtcggtatagtggctacgtttactacgcagactcagtgaagggc

SEQ ID NO: 193 - DNA, 51 bp, synthetic construct
  misc_feature 1..51: note = N-HCDR2-3
  source 1..51: mol_type = other DNA
tccattagtcgggctagtagctacgtttactacgcagactcagtgaagggc

SEQ ID NO: 194 - DNA, 51 bp, synthetic construct
  misc_feature 1..51: note = N-HCDR2-4
  source 1..51: mol_type = other DNA
tccattagtcggtatagtggctacatatactacgcagactcagtgaagggc

SEQ ID NO: 195 - DNA, 51 bp, synthetic construct
  misc_feature 1..51: note = N-HCDR2-5
  source 1..51: mol_type = other DNA
tccattagtgctaggagtcgttaccactactacgcagactcagtgaagggc

SEQ ID NO: 196 - DNA, 51 bp, synthetic construct
  misc_feature 1..51: note = N-HCDR2-6
  source 1..51: mol_type = other DNA
tccattagtgctcgtagtagttacatatactacgcagactcagtgaagggc

SEQ ID NO: 197 - DNA, 51 bp, synthetic construct
  misc_feature 1..51: note = N-HCDR2-7
  source 1..51: mol_type = other DNA
tccattagtgctcttagtagttacatatactacgcagactcagtgaggggc

SEQ ID NO: 198 - DNA, 51 bp, synthetic construct
  misc_feature 1..51: note = N-HCDR2-8
  source 1..51: mol_type = other DNA
tccattagtgctcagagtagtcacatatactacgcagactcagtggagggc

SEQ ID NO: 199 - DNA, 51 bp, synthetic construct
  misc_feature 1..51: note = N-HCDR2-9
  source 1..51: mol_type = other DNA
tccattagtgctcggagtagctacctatactacgcagactcagtgaagggc

SEQ ID NO: 200 - DNA, 51 bp, synthetic construct
  misc_feature 1..51: note = N-HCDR2-10
  source 1..51: mol_type = other DNA
tccattagtgctcggagtagctacatatactacgcagactcagtgaagggc

SEQ ID NO: 201 - DNA, 51 bp, synthetic construct
  misc_feature 1..51: note = N-HCDR2-11
  source 1..51: mol_type = other DNA
tccattagtgctcgcagtagctaccgctactacgcagactcagtgaagggc

SEQ ID NO: 202 - DNA, 51 bp, synthetic construct
  misc_feature 1..51: note = N-HCDR2-12
  source 1..51: mol_type = other DNA
tccattagtgctcggagtagctacatctactacgcagattcagtgaagggc

SEQ ID NO: 203 - DNA, 51 bp, synthetic construct
  misc_feature 1..51: note = N-HCDR2-13
  source 1..51: mol_type = other DNA
tccattagtgctcggagtagctaccgctactacgcagattcagtgaagggc

SEQ ID NO: 204 - DNA, 51 bp, synthetic construct
  misc_feature 1..51: note = N-HCDR2-14
  source 1..51: mol_type = other DNA
tccattagtgctcggagtagctacatctactacgcaggttcagtgaagggc

SEQ ID NO: 205 - DNA, 51 bp, synthetic construct
  misc_feature 1..51: note = N-HCDR2-15
  source 1..51: mol_type = other DNA
tccattagttctaggagtagccaccaatactacgcaggttcagtgaagggc

SEQ ID NO: 206 - DNA, 51 bp, synthetic construct
  misc_feature 1..51: note = N-HCDR2-16
  source 1..51: mol_type = other DNA
tccattagtgctaggagtagctacatctactacgcagattcagtgaagggc

SEQ ID NO: 207 - DNA, 51 bp, synthetic construct
  misc_feature 1..51: note = N-HCDR2-17
  source 1..51: mol_type = other DNA
tccattagtgctctgagtagctaccgatactacgcagattcagtgaagggc

SEQ ID NO: 208 - DNA, 51 bp, synthetic construct
  misc_feature 1..51: note = N-HCDR2-18
  source 1..51: mol_type = other DNA
tccattagtagtagtagtagttacatatactacgcagactcagtgaagggc

SEQ ID NO: 209 - DNA, 21 bp, synthetic construct
  misc_feature 1..21: note = N-HCDR3-1
  source 1..21: mol_type = other DNA
gatattggcggtatggacgtc

SEQ ID NO: 210 - DNA, 30 bp, synthetic construct
  misc_feature 1..30: note = N-HCDR3-2
  source 1..30: mol_type = other DNA
cttgctacgaggcataatgcttttgatatc

SEQ ID NO: 211 - DNA, 30 bp, synthetic construct
  misc_feature 1..30: note = N-HCDR3-3
  source 1..30: mol_type = other DNA
cttgctacgaggaataatgcttttgatatc

SEQ ID NO: 212 - DNA, 30 bp, synthetic construct
  misc_feature 1..30: note = N-HCDR3-4
  source 1..30: mol_type = other DNA
cttgctacgaggcgtgatgcttttgatatc

SEQ ID NO: 213 - DNA, 30 bp, synthetic construct
  misc_feature 1..30: note = N-HCDR3-5
  source 1..30: mol_type = other DNA
cttgctacgaggcaaaacgcttttgatatc

SEQ ID NO: 214 - DNA, 30 bp, synthetic construct
  misc_feature 1..30: note = N-HCDR3-6
  source 1..30: mol_type = other DNA
cttgctaccaggcatgtcgcttttgatatc

SEQ ID NO: 215 - DNA, 30 bp, synthetic construct
  misc_feature 1..30: note = N-HCDR3-7
  source 1..30: mol_type = other DNA
cttgctaccaggcatggcgcttttgatatc

SEQ ID NO: 216 - DNA, 30 bp, synthetic construct
  misc_feature 1..30: note = N-HCDR3-8
  source 1..30: mol_type = other DNA
cttgctaccaggcataacgcttttgatatc

SEQ ID NO: 217 - DNA, 30 bp, synthetic construct
  misc_feature 1..30: note = N-HCDR3-9
  source 1..30: mol_type = other DNA
cttgctaccaggcatctcgcttttgatatc

SEQ ID NO: 218 - DNA, 30 bp, synthetic construct
  misc_feature 1..30: note = N-HCDR3-10
  source 1..30: mol_type = other DNA
cttgctaccaggcatagcgcttttgatatc

SEQ ID NO: 219 - DNA, 30 bp, synthetic construct
  misc_feature 1..30: note = N-HCDR3-11
  source 1..30: mol_type = other DNA
cttgctaccaggcgcgacgcttttgatatc

SEQ ID NO: 220 - DNA, 30 bp, synthetic construct
  misc_feature 1..30: note = N-HCDR3-12
  source 1..30: mol_type = other DNA
cttgctaccaggcacagcgcttttgatatc

SEQ ID NO: 221 - DNA, 30 bp, synthetic construct
  misc_feature 1..30: note = N-HCDR3-13
  source 1..30: mol_type = other DNA
cttggtaccaggcgcgtcgcttttgatatc

SEQ ID NO: 222 - DNA, 30 bp, synthetic construct
  misc_feature 1..30: note = N-HCDR3-14
  source 1..30: mol_type = other DNA
cttggtctcaggcacgacgcttttgatatc

SEQ ID NO: 223 - DNA, 30 bp, synthetic construct
  misc_feature 1..30: note = N-HCDR3-15
  source 1..30: mol_type = other DNA
cttgctaccaggcgcatcgcttttgatatc

SEQ ID NO: 224 - DNA, 30 bp, synthetic construct
  misc_feature 1..30: note = N-HCDR3-16
  source 1..30: mol_type = other DNA
cttgctaccaggcgcgtcgcttttgatatc

SEQ ID NO: 225 - DNA, 30 bp, synthetic construct
  misc_feature 1..30: note = N-HCDR3-17
  source 1..30: mol_type = other DNA
cttggtacgaggcatgatgcttttgatatc

SEQ ID NO: 226 - protein, 270 aa, Homo sapiens
MKPKMKYSTNKISTAKWKNTASKALCFKLGKSQQKAKEVCPMYFMKLRSGLMIKKEACYFRRETTKRPSLKTGRKHKRHLVLAACQQQSTVECFAFGISGVQKYTRALHDSSITGISPITEYLASLSTYNDQSITFALEDESYEIYVEDLKKDEKKDKVLLSYYESQHPSNESGDGVDGKMLMVTLSPTKDFWLHANNKEHSVELHKCEKPLPDQAFFVLHNMHSNCVSFECKTDPGVFIGVKDNHLALIKVDSSENLCTENILFKLSET

SEQ ID NO: 227 - protein, 269 aa, Macaca fascicularis
MKPKMKYSTNKISTAKRKNTASKALCFKLGKSQQKAKEVCHVYFMKLRSGLMIKKEACYFRRETTKRPSLKTGGKHKGHLVLAACQQQSTVECFAFGISGVPKYTRALHDSSITGISPITESLASLSTYNDQSITFALEDESYEIYVEDLKKDKKKDKVLLSYYESQHPSSESGDGVDGKMLMVTLSPTKDFWLQANNKEHSVELHKCEKPLPDQAFFVLHNRSFNCVSFECKTDPGVFIGVKDNHLALIKVDYSENLGSENILFKLSE

SEQ ID NO: 228 - DNA, 645 bp, synthetic construct
  misc_feature 1..645: note = N-LC-1
  source 1..645: mol_type = other DNA
cagtctgtgctgactcagccaccctcagcgtctgggacccccgggcagagggtcaccatctcctgcactgggagcagctccaacatcggggcagtttatgatgtacactggtatcagcagctcccaggaacggcccccaaactcctcatctataggaataatcagcggccctcaggggtccctgaccgattctctggctccaagtctggcacctcagcctccctggccatcagtgggctccggtccgaggatgaggctgattattactgccagacttatgacagcagccgttgggtgttcggcggaggaaccaagctgacggtcctaggtcaacccaaggccgctcccagcgtgaccctgttcccccccagcagcgaggagctgcaggccaacaaggccaccctggtgtgtctgatcagcgacttctacccaggcgccgtgaccgtggcctggaaggccgacagcagccccgtgaaggccggcgtggagaccaccacccccagcaagcagagcaacaacaagtacgccgccagcagctacctgagcctgaccccagagcagtggaagagccacaggagctacagctgccaggtcacccacgagggcagcaccgtggaaaagaccgtggccccaaccgagtgctcc

SEQ ID NO: 229 - DNA, 645 bp, synthetic construct
  misc_feature 1..645: note = N-LC-2
  source 1..645: mol_type = other DNA
cagtctgtgctgactcagccaccctcagcgtctgggacccccgggcagagggtcaccatctcctgcactgggagcagctccaacatcggggcagtttatgatgtacactggtatcagcagctcccaggaacggcccccaaactcctcatctataggaataatcagcggccctcaggggtccctgaccgattctctggctccaagtctggcacctcagcctccctggccatcagtgggctccggtccgaggatgaggctgattattactgccagtcctatgacagcagccgttgggtgttcggcggaggaaccaagctgacggtcctaggtcaacccaaggccgctcccagcgtgaccctgttcccccccagcagcgaggagctgcaggccaacaaggccaccctggtgtgtctgatcagcgacttctacccaggcgccgtgaccgtggcctggaaggccgacagcagccccgtgaaggccggcgtggagaccaccacccccagcaagcagagcaacaacaagtacgccgccagcagctacctgagcctgaccccagagcagtggaagagccacaggagctacagctgccaggtcacccacgagggcagcaccgtggaaaagaccgtggccccaaccgagtgctcc

SEQ ID NO: 230 - DNA, 645 bp, synthetic construct
  misc_feature 1..645: note = N-LC-3
  source 1..645: mol_type = other DNA
cagtctgtgctgactcagccaccctcagcgtctgggacccccgggcagagggtcaccatctcctgcactgggagcagctccaacatcggggcagtttataatgtacactggtatcagcagctcccaggaacggcccccaaactcctcatctataggaataatcagcggccctcaggggtccctgaccgattctctggctccaagtctggcacctcagcctccctggccatcagtgggctccggtccgaggatgaggctgattattactgccagtcctatgacagcagccgttgggtgttcggcggaggaaccaagctgacggtcctaggtcaacccaaggccgctcccagcgtgaccctgttcccccccagcagcgaggagctgcaggccaacaaggccaccctggtgtgtctgatcagcgacttctacccaggcgccgtgaccgtggcctggaaggccgacagcagccccgtgaaggccggcgtggagaccaccacccccagcaagcagagcaacaacaagtacgccgccagcagctacctgagcctgaccccagagcagtggaagagccacaggagctacagctgccaggtcacccacgagggcagcaccgtggaaaagaccgtggccccaaccgagtgctcc

SEQ ID NO: 231 - DNA, 645 bp, synthetic construct
  misc_feature 1..645: note = N-LC-4
  source 1..645: mol_type = other DNA
cagtctgtgctgactcagccaccctcagcgtctgggacccccgggcagagggtcaccatctcctgcactgggagcagctccaacatcggggcagtttataatgtacactggtatcagcagctcccaggaacggcccccaaactcctcatctataggaataatcagcggccctcaggggtccctgaccgattctctggctccaagtctggcacctcagcctccctggccatcagtgggctccggtccgaggatgaggctgattattactgccagtcctatgacagccgccgttgggtgttcggcggaggaaccaagctgacggtcctaggtcaacccaaggccgctcccagcgtgaccctgttcccccccagcagcgaggagctgcaggccaacaaggccaccctggtgtgtctgatcagcgacttctacccaggcgccgtgaccgtggcctggaaggccgacagcagccccgtgaaggccggcgtggagaccaccacccccagcaagcagagcaacaacaagtacgccgccagcagctacctgagcctgaccccagagcagtggaagagccacaggagctacagctgccaggtcacccacgagggcagcaccgtggaaaagaccgtggccccaaccgagtgctcc

SEQ ID NO: 232 - DNA, 648 bp, synthetic construct
  misc_feature 1..648: note = N-LC-5
  source 1..648: mol_type = other DNA
cagtctgtgctgactcagccaccctcagcgtctgggacccccgggcagagggtcacgatatcctgttctggaagcagctccaacatcggaaataatgctgtaagctggtatcagcagctcccaggaacggcccccaaactcctcatctatgccagtaacatgagagtcattggggtccctgaccgattctctggctccaagtctggcacctcagcctccctggccatcagtgggctccggtccgaggatgaggctgattattactgtggagcatgggatgacagccagaaggctcttgttttcggcggaggaaccaagcttacggtcctaggtcaacccaaggccgctcccagcgtgaccctgttcccccccagcagcgaggagctgcaggccaacaaggccaccctggtgtgtctgatcagcgacttctacccaggcgccgtgaccgtggcctggaaggccgacagcagccccgtgaaggccggcgtggagaccaccacccccagcaagcagagcaacaacaagtacgccgccagcagctacctgagcctgaccccagagcagtggaagagccacaggagctacagctgccaggtcacccacgagggcagcaccgtggaaaagaccgtggccccaaccgagtgctcc

SEQ ID NO: 233 - DNA, 648 bp, synthetic construct
  misc_feature 1..648: note = N-LC-6
  source 1..648: mol_type = other DNA
cagtctgtgctgactcagccaccctcagcgtctgggacccccgggcagagggtcacgatatcctgttctggaagcagctccaacatcggacgtaatgctgtaaactggtatcagcagctcccaggaacggcccccaaactcctcatctatgccagtaacatgagagtcattggggtccctgaccgattctctggctccaagtctggcacctcagcctccctggccatcagtgggctccggtccgaggatgaggctgattattactgtgcagcatgggatgacagccagaaggcttgggttttcggcggaggaaccaagcttacggtcctaggtcaacccaaggccgctcccagcgtgaccctgttcccccccagcagcgaggagctgcaggccaacaaggccaccctggtgtgtctgatcagcgacttctacccaggcgccgtgaccgtggcctggaaggccgacagcagccccgtgaaggccggcgtggagaccaccacccccagcaagcagagcaacaacaagtacgccgccagcagctacctgagcctgaccccagagcagtggaagagccacaggagctacagctgccaggtcacccacgagggcagcaccgtggaaaagaccgtggccccaaccgagtgctcc

SEQ ID NO: 234 - DNA, 648 bp, synthetic construct
  misc_feature 1..648: note = N-LC-7
  source 1..648: mol_type = other DNA
cagtctgtgctgactcagccaccctcagcgtctgggacccccgggcagagggtcacgatatcctgttctggaagcagctccaacatcggacgtaatgctgtaaactggtatcagcagctcccaggaacggcccccaaactcctcatctatgccagtaacatgagagtcttaggggtccctgaccgattctctggctccaagtctggcacctcagcctccctggccatcagtgggctccggtccgaggatgaggctgattattactgttgggcatgggatgacagccagaaggctgtggttttcggcggaggaaccaagcttacggtcctaggtcaacccaaggccgctcccagcgtgaccctgttcccccccagcagcgaggagctgcaggccaacaaggccaccctggtgtgtctgatcagcgacttctacccaggcgccgtgaccgtggcctggaaggccgacagcagccccgtgaaggccggcgtggagaccaccacccccagcaagcagagcaacaacaagtacgccgccagcagctacctgagcctgaccccagagcagtggaagagccacaggagctacagctgccaggtcacccacgagggcagcaccgtggaaaagaccgtggccccaaccgagtgctcc

SEQ ID NO: 235 - DNA, 648 bp, synthetic construct
  misc_feature 1..648: note = N-LC-8
  source 1..648: mol_type = other DNA
cagtctgtgctgactcagccaccctcagcgtctgggacccccgggcagagggtcacgatatcctgttctggaagctgctccaacatcggacgtaatgctgtaaactggtatcagcagctcccaggaacggcccccaaactcctcatctatgccagtaacatgagagtcataggggtccctgaccgattctctggctccaagtctggcacctcagcctccctggccatcagtgggctccggtccgaggatgaggctgattattactgtgaggcatgggatgacagccagaagggtgtggttttcggcggaggaaccaagcttacggtcctaggtcaacccaaggccgctcccagcgtgaccctgttcccccccagcagcgaggagctgcaggccaacaaggccaccctggtgtgtctgatcagcgacttctacccaggcgccgtgaccgtggcctggaaggccgacagcagccccgtgaaggccggcgtggagaccaccacccccagcaagcagagcaacaacaagtacgccgccagcagctacctgagcctgaccccagagcagtggaagagccacaggagctacagctgccaggtcacccacgagggcagcaccgtggaaaagaccgtggccccaaccgagtgctcc

SEQ ID NO: 236 - DNA, 648 bp, synthetic construct
  misc_feature 1..648: note = N-LC-9
  source 1..648: mol_type = other DNA
cagtctgtgctgactcagccaccctcagcgtctgggacccccgggcagagggtcacgatatcctgttctggaagcagctccaacatcggacgtaatgctgtaaactggtatcagcagctcccaggaacggcccccaaactcctcatctatgccagtaacatgagagtcattggggtccctgaccgattctctggctccaagtctggcacctcagcctccctggccatcagtgggctccggtccgaggatgaggctgattattactgtggagcatgggatgacagccagaagcgttatgttttcggcggaggaaccaagcttacggtcctaggtcaacccaaggccgctcccagcgtgaccctgttcccccccagcagcgaggagctgcaggccaacaaggccaccctggtgtgtctgatcagcgacttctacccaggcgccgtgaccgtggcctggaaggccgacagcagccccgtgaaggccggcgtggagaccaccacccccagcaagcagagcaacaacaagtacgccgccagcagctacctgagcctgaccccagagcagtggaagagccacaggagctacagctgccaggtcacccacgagggcagcaccgtggaaaagaccgtggccccaaccgagtgctcc

SEQ ID NO: 237 - DNA, 648 bp, synthetic construct
  misc_feature 1..648: note = N-LC-10
  source 1..648: mol_type = other DNA
cagtctgtgctgactcagccaccctcagcgtctgggacccccgggcagagggtcacgatatcctgttctggaagcagctccaacatcggaaataatgctgtaaactggtatcagcagctcccaggaacggcccccaaactcctcatctatgccagtaacatgagaggctctggggtccctgaccgattctctggctccaagtctggcacctcagcctccctggccatcagtgggctccggtccgaggatgaggctgattattactgtgcggcatgggatgacagccagaagggtcaggttttcggcggaggaaccaagcttacggtcctaggtcaacccaaggccgctcccagcgtgaccctgttcccccccagcagcgaggagctgcaggccaacaaggccaccctggtgtgtctgatcagcgacttctacccaggcgccgtgaccgtggcctggaaggccgacagcagccccgtgaaggccggcgtggagaccaccacccccagcaagcagagcaacaacaagtacgccgccagcagctacctgagcctgaccccagagcagtggaagagccacaggagctacagctgccaggtcacccacgagggcagcaccgtggaaaagaccgtggccccaaccgagtgctcc

SEQ ID NO: 238 - DNA, 648 bp, synthetic construct
  misc_feature 1..648: note = N-LC-11
  source 1..648: mol_type = other DNA
cagtctgtgctgactcagccaccctcagcgtctgggacccccgggcagagggtcacgatatcctgttctggaagcagctccaacatcggaagtaatgctgtaagctggtatcagcagctcccaggaacggcccccaaactcctcatctatgccagtaacatgagaggctctggggtccctgaccgattctctggctccaagtctggcacctcagcctccctggccatcagtgggctccggtccgaggatgaggctgattattactgtgcagcatgggatgacagccagaaggttgtggttttcggcggaggaaccaagcttacggtcctaggtcaacccaaggccgctcccagcgtgaccctgttcccccccagcagcgaggagctgcaggccaacaaggccaccctggtgtgtctgatcagcgacttctacccaggcgccgtgaccgtggcctggaaggccgacagcagccccgtgaaggccggcgtggagaccaccacccccagcaagcagagcaacaacaagtacgccgccagcagctacctgagcctgaccccagagcagtggaagagccacaggagctacagctgccaggtcacccacgagggcagcaccgtggaaaagaccgtggccccaaccgagtgctcc

SEQ ID NO: 239 - DNA, 648 bp, synthetic construct
  misc_feature 1..648: note = N-LC-12
  source 1..648: mol_type = other DNA
cagtctgtgctgactcagccaccctcagcgtctgggacccccgggcagagggtcacgatatcctgttctggaagcagctccaacatcggacgtaatgctgtaaactggtatcagcagctcccaggaacggcccccaaactcctcatctatgccagtaacatgagagtctctggggtccctgaccgattctctggctccaagtctggcacctcagcctccctggccatcagtgggctccggtccgaggatgaggctgattattactgttgggcatgggatgacagccagaaggttggtgttttcggcggaggaaccaagcttacggtcctaggtcaacccaaggccgctcccagcgtgaccctgttcccccccagcagcgaggagctgcaggccaacaaggccaccctggtgtgtctgatcagcgacttctacccaggcgccgtgaccgtggcctggaaggccgacagcagccccgtgaaggccggcgtggagaccaccacccccagcaagcagagcaacaacaagtacgccgccagcagctacctgagcctgaccccagagcagtggaagagccacaggagctacagctgccaggtcacccacgagggcagcaccgtggaaaagaccgtggccccaaccgagtgctcc

SEQ ID NO: 240 - DNA, 648 bp, synthetic construct
  misc_feature 1..648: note = N-LC-13
  source 1..648: mol_type = other DNA
cagtctgtgctgactcagccaccctcagcgtctgggacccccgggcagagggtcacgatatcctgttctggaagcagctccaacatcggaaataatgctgtaaactggtatcagcagctcccaggaacggcccccaaactcctcatctatgccagtaacatgagaggcttaggggtccctgaccgattctctggctccaagtctggcacctcagcctccctggccatcagtgggctccggtccgaggatgaggctgattattactgtggggcatgggatgacagccagaaggtttttgttttcggcggaggaaccaagcttacggtcctaggtcaacccaaggccgctcccagcgtgaccctgttcccccccagcagcgaggagctgcaggccaacaaggccaccctggtgtgtctgatcagcgacttctacccaggcgccgtgaccgtggcctggaaggccgacagcagccccgtgaaggccggcgtggagaccaccacccccagcaagcagagcaacaacaagtacgccgccagcagctacctgagcctgaccccagagcagtggaagagccacaggagctacagctgccaggtcacccacgagggcagcaccgtggaaaagaccgtggccccaaccgagtgctcc

SEQ ID NO: 241 - DNA, 648 bp, synthetic construct
  misc_feature 1..648: note = N-LC-14
  source 1..648: mol_type = other DNA
cagtctgtgctgactcagccaccctcagcgtctgggacccccgggcagagggtcacgatatcctgttctggaagcagctccaacatcggacgtaatgctgtaaactggtatcagcagctcccaggaacggcccccaaactcctcatctatgccagtaacatgagacgctctggggtccctgaccgattctctggctccaagtctggcacctcagcctccctggccatcagtgggctccggtccgaggatgaggctgattattactgttcagcatgggatgacagccagaaggttgtggttttcggcggaggaaccaagcttacggtcctaggtcaacccaaggccgctcccagcgtgaccctgttcccccccagcagcgaggagctgcaggccaacaaggccaccctggtgtgtctgatcagcgacttctacccaggcgccgtgaccgtggcctggaaggccgacagcagccccgtgaaggccggcgtggagaccaccacccccagcaagcagagcaacaacaagtacgccgccagcagctacctgagcctgaccccagagcagtggaagagccacaggagctacagctgccaggtcacccacgagggcagcaccgtggaaaagaccgtggccccaaccgagtgctcc

SEQ ID NO: 242 - DNA, 648 bp, synthetic construct
  misc_feature 1..648: note = N-LC-15
  source 1..648: mol_type = other DNA
cagtctgtgctgactcagccaccctcagcgtctgggacccccgggcagagggtcacgatatcctgttctggaagcagctccaacatcggaaataatgctgtaaactggtatcagcagctcccaggaacggcccccaaactcctcatctatgccagtaacatgagacgcccgggggtccctgaccgattctctggctccaagtctggcacctcagcctccctggccatcagtgggctccggtccgaggatgaggctgattattactgtgaggcatgggatgacagccagaaggctgttgttttcggcggaggaaccaagcttacggtcctaggtcaacccaaggccgctcccagcgtgaccctgttcccccccagcagcgaggagctgcaggccaacaaggccaccctggtgtgtctgatcagcgacttctacccaggcgccgtgaccgtggcctggaaggccgacagcagccccgtgaaggccggcgtggagaccaccacccccagcaagcagagcaacaacaagtacgccgccagcagctacctgagcctgaccccagagcagtggaagagccacaggagctacagctgccaggtcacccacgagggcagcaccgtggaaaagaccgtggccccaaccgagtgctcc

SEQ ID NO: 243 - DNA, 648 bp, synthetic construct
  misc_feature 1..648: note = N-LC-16
  source 1..648: mol_type = other DNA
cagtctgtgctgactcagccaccctcagcgtctgggacccccgggcagagggtcacgatatcctgttctggaagcagctccaacatcggaaataatgctgtaaactggtatcagcagctcccaggaacggcccccaaactcctcatctatgccagtaacatgagacgcatgggggtccctgaccgattctctggctccaagtctggcacctcagcctccctggccatcagtgggctccggtccgaggatgaggctgattattactgtgcggcatgggatgacagccagaaggcttttgttttcggcggaggaaccaagcttacggtcctaggtcaacccaaggccgctcccagcgtgaccctgttcccccccagcagcgaggagctgcaggccaacaaggccaccctggtgtgtctgatcagcgacttctacccaggcgccgtgaccgtggcctggaaggccgacagcagccccgtgaaggccggcgtggagaccaccacccccagcaagcagagcaacaacaagtacgccgccagcagctacctgagcctgaccccagagcagtggaagagccacaggagctacagctgccaggtcacccacgagggcagcaccgtggaaaagaccgtggccccaaccgagtgctcc

SEQ ID NO: 244 - DNA, 648 bp, synthetic construct
  misc_feature 1..648: note = N-LC-17
  source 1..648: mol_type = other DNA
cagtctgtgctgactcagccaccctcagcgtctgggacccccgggcagagggtcacgatatcctgttctggaagcagctccaacatcggaaataatgctgtaaactggtatcagcagctcccaggaacggcccccaaactcctcatctatgccagtaacatgagacgcctgggggtccctgaccgattctctggctccaagtctggcacctcagcctccctggccatcagtgggctccggtccgaggatgaggctgattattactgtgcggcatgggatgacagccagaaggcttgggttttcggcggaggaaccaagcttacggtcctaggtcaacccaaggccgctcccagcgtgaccctgttcccccccagcagcgaggagctgcaggccaacaaggccaccctggtgtgtctgatcagcgacttctacccaggcgccgtgaccgtggcctggaaggccgacagcagccccgtgaaggccggcgtggagaccaccacccccagcaagcagagcaacaacaagtacgccgccagcagctacctgagcctgaccccagagcagtggaagagccacaggagctacagctgccaggtcacccacgagggcagcaccgtggaaaagaccgtggccccaaccgagtgctcc

SEQ ID NO: 245 - DNA, 648 bp, synthetic construct
  misc_feature 1..648: note = N-LC-18
  source 1..648: mol_type = other DNA
cagtctgtgctgactcagccaccctcagcgtctgggacccccgggcagagggtcacgatatcctgttctggaagcagctccaacatcggaaataatgctgtaaactggtatcagcagctcccaggaacggcccccaaactcctcatctatgccagtaacatgagacgcccgggggtccctgaccgattctctggctccaagtctggcacctcagcctccctggccatcagtgggctccggtccgaggatgaggctgattattactgtgcggcatgggatgacagccagaaggtttttgttttcggcggaggaaccaagcttacggtcctaggtcaacccaaggccgctcccagcgtgaccctgttcccccccagcagcgaggagctgcaggccaacaaggccaccctggtgtgtctgatcagcgacttctacccaggcgccgtgaccgtggcctggaaggccgacagcagccccgtgaaggccggcgtggagaccaccacccccagcaagcagagcaacaacaagtacgccgccagcagctacctgagcctgaccccagagcagtggaagagccacaggagctacagctgccaggtcacccacgagggcagcaccgtggaaaagaccgtggccccaaccgagtgctcc

SEQ ID NO: 246 - DNA, 648 bp, synthetic construct
  misc_feature 1..648: note = N-LC-19
  source 1..648: mol_type = other DNA
cagtctgtgctgactcagccaccctcagcgtctgggacccccgggcagagggtcacgatatcctgttctggaagcagctccaacatcggaaataatgctgtaaactggtatcagcagctcccaggaacggcccccaaactcctcatctatgccagtaacatgagacgcctgggggtccctgaccgattctctggctccaagtctggcacctcagcctccctggccatcagtgggctccggtccgaggatgaggctgattattactgtggggcatgggatgacagccagaaggcttttgttttcggcggaggaaccaagcttacggtcctaggtcaacccaaggccgctcccagcgtgaccctgttcccccccagcagcgaggagctgcaggccaacaaggccaccctggtgtgtctgatcagcgacttctacccaggcgccgtgaccgtggcctggaaggccgacagcagccccgtgaaggccggcgtggagaccaccacccccagcaagcagagcaacaacaagtacgccgccagcagctacctgagcctgaccccagagcagtggaagagccacaggagctacagctgccaggtcacccacgagggcagcaccgtggaaaagaccgtggccccaaccgagtgctcc

SEQ ID NO: 247 - DNA, 648 bp, synthetic construct
  misc_feature 1..648: note = N-LC-20
  source 1..648: mol_type = other DNA
cagtctgtgctgactcagccaccctcagcgtctgggacccccgggcagagggtcacgatatcctgttctggaagcagctccaacatcggacgcaatgctgtaagctggtatcagcagctcccaggaacggcccccaaactcctcatctatgccagtaacatgagacgtctgggggtccctgaccgattctctggctccaagtctggcacctcagcctccctggccatcagtgggctccggtccgaggatgaggctgattattactgttgggcatgggatgacagccagaaggctgttgttttcggcggaggaaccaagcttacggtcctaggtcaacccaaggccgctcccagcgtgaccctgttcccccccagcagcgaggagctgcaggccaacaaggccaccctggtgtgtctgatcagcgacttctacccaggcgccgtgaccgtggcctggaaggccgacagcagccccgtgaaggccggcgtggagaccaccacccccagcaagcagagcaacaacaagtacgccgccagcagctacctgagcctgaccccagagcagtggaagagccacaggagctacagctgccaggtcacccacgagggcagcaccgtggaaaagaccgtggccccaaccgagtgctcc

SEQ ID NO: 248 - DNA, 648 bp, synthetic construct
  misc_feature 1..648: note = N-LC-21
  source 1..648: mol_type = other DNA
cagtctgtgctgactcagccaccctcagcgtctgggacccccgggcagagggtcacgatatcctgttctggaagcagctccaacatcggacacaatgctgtaagctggtatcagcagctcccaggaacggcccccaaactcctcatctatgccagtaacatgagacgtctgggggtccctgaccgattctctggctccaagtctggcacctcagcctccctggccatcagtgggctccggtccgaggatgaggctgattattactgtggggcatgggatgacagccagaaggttgtggttttcggcggaggaaccaagcttacggtcctaggtcaacccaaggccgctcccagcgtgaccctgttcccccccagcagcgaggagctgcaggccaacaaggccaccctggtgtgtctgatcagcgacttctacccaggcgccgtgaccgtggcctggaaggccgacagcagccccgtgaaggccggcgtggagaccaccacccccagcaagcagagcaacaacaagtacgccgccagcagctacctgagcctgaccccagagcagtggaagagccacaggagctacagctgccaggtcacccacgagggcagcaccgtggaaaagaccgtggccccaaccgagtgctcc

SEQ ID NO: 249 - DNA, 648 bp, synthetic construct
  misc_feature 1..648: note = N-LC-22
  source 1..648: mol_type = other DNA
cagtctgtgctgactcagccaccctcagcgtctgggacccccgggcagagggtcacgatatcctgttctggaagcagctccaacatcggacgcaatgctgtaaactggtatcagcagctcccaggaacggcccccaaactcctcatctatgccagtaacatgagaggtatgggggtccctgaccgattctctggctccaagtctggcacctcagcctccctggccatcagtgggctccggtccgaggatgaggctgattattactgttcggcatgggatgacagccagaaggttgttgttttcggcggaggaaccaagcttacggtcctaggtcaacccaaggccgctcccagcgtgaccctgttcccccccagcagcgaggagctgcaggccaacaaggccaccctggtgtgtctgatcagcgacttctacccaggcgccgtgaccgtggcctggaaggccgacagcagccccgtgaaggccggcgtggagaccaccacccccagcaagcagagcaacaacaagtacgccgccagcagctacctgagcctgaccccagagcagtggaagagccacaggagctacagctgccaggtcacccacgagggcagcaccgtggaaaagaccgtggccccaaccgagtgctcc

SEQ ID NO: 250 - DNA, 648 bp, synthetic construct
  misc_feature 1..648: note = N-LC-23
  source 1..648: mol_type = other DNA
cagtctgtgctgactcagccaccctcagcgtctgggacccccgggcagagggtcacgatatcctgttctggaagcagctccaacatcggacacaatgctgtatggtggtatcagcagctcccaggaacggcccccaaactcctcatctatgccagtaacatgagacgtatgggggtccctgaccgattctctggctccaagtctggcacctcagcctccctggccatcagtgggctccggtccgaggatgaggctgattattactgtgcggcatgggatgacagccagaaggctgttgttttcggcggaggaaccaagcttacggtcctaggtcaacccaaggccgctcccagcgtgaccctgttcccccccagcagcgaggagctgcaggccaacaaggccaccctggtgtgtctgatcagcgacttctacccaggcgccgtgaccgtggcctggaaggccgacagcagccccgtgaaggccggcgtggagaccaccacccccagcaagcagagcaacaacaagtacgccgccagcagctacctgagcctgaccccagagcagtggaagagccacaggagctacagctgccaggtcacccacgagggcagcaccgtggaaaagaccgtggccccaaccgagtgctcc

SEQ ID NO: 251 - DNA, 648 bp, synthetic construct
  misc_feature 1..648: note = N-LC-24
  source 1..648: mol_type = other DNA
cagtctgtgctgactcagccaccctcagcgtctgggacccccgggcagagggtcacgatatcctgttctggaagcagctccaacatcggacgcaatgctgtaaactggtatcagcagctcccaggaacggcccccaaactcctcatctatgccagtaacatgagacgtccgggggtccctgaccgattctctggctccaagtctggcacctcagcctccctggccatcagtgggctccggtccgaggatgaggctgattattactgttcggcatgggatgacagccagaaggctggggttttcggcggaggaaccaagcttacggtcctaggtcaacccaaggccgctcccagcgtgaccctgttcccccccagcagcgaggagctgcaggccaacaaggccaccctggtgtgtctgatcagcgacttctacccaggcgccgtgaccgtggcctggaaggccgacagcagccccgtgaaggccggcgtggagaccaccacccccagcaagcagagcaacaacaagtacgccgccagcagctacctgagcctgaccccagagcagtggaagagccacaggagctacagctgccaggtcacccacgagggcagcaccgtggaaaagaccgtggccccaaccgagtgctcc

SEQ ID NO: 252 - DNA, 648 bp, synthetic construct
  misc_feature 1..648: note = N-LC-25
  source 1..648: mol_type = other DNA
cagtctgtgctgactcagccaccctcagcgtctgggacccccgggcagagggtcacgatatcctgttctggaagcagctccaacatcggaaataatgctgtaaactggtatcagcagctcccaggaacggcccccaaactcctcatctatgccagtaacatgagacgcttaggggtccctgaccgattctctggctccaagtctggcacctcagcctccctggccatcagtgggctccggtccgaggatgaggctgattattactgtgcggcatgggatgacagccagaaggctttggttttcggcggaggaaccaagcttacggtcctaggtcaacccaaggccgctcccagcgtgaccctgttcccccccagcagcgaggagctgcaggccaacaaggccaccctggtgtgtctgatcagcgacttctacccaggcgccgtgaccgtggcctggaaggccgacagcagccccgtgaaggccggcgtggagaccaccacccccagcaagcagagcaacaacaagtacgccgccagcagctacctgagcctgaccccagagcagtggaagagccacaggagctacagctgccaggtcacccacgagggcagcaccgtggaaaagaccgtggccccaaccgagtgctcc

SEQ ID NO: 253 - DNA, 648 bp, synthetic construct
  misc_feature 1..648: note = N-LC-26
  source 1..648: mol_type = other DNA
cagtctgtgctgactcagccaccctcagcgtctgggacccccgggcagagggtcacgatatcctgttctggaagcagctccaacatcggaaataatgctgtaaactggtatcagcagctcccaggaacggcccccaaactcctcatctatgccagtaacatgagacgcttaggggtccctgaccgattctctggctccaagtctggcacctcagcctccctggccatcagtgggctccggtccgaggatgaggctgattattactgtgcagcatgggatgacagccagaaggctgttgttttcggcggaggaaccaagcttacggtcctaggtcaacccaaggccgctcccagcgtgaccctgttcccccccagcagcgaggagctgcaggccaacaaggccaccctggtgtgtctgatcagcgacttctacccaggcgccgtgaccgtggcctggaaggccgacagcagccccgtgaaggccggcgtggagaccaccacccccagcaagcagagcaacaacaagtacgccgccagcagctacctgagcctgaccccagagcagtggaagagccacaggagctacagctgccaggtcacccacgagggcagcaccgtggaaaagaccgtggccccaaccgagtgctcc

SEQ ID NO: 254 - DNA, 1338 bp, synthetic construct
  misc_feature 1..1338: note = N-HC-1
  source 1..1338: mol_type = other DNA
gaggtgcagctgttggagtctgggggaggcttggtacagcctggggggtccctgagactctcctgtgcagcctctggattcaccttcagtgactactacatgaactgggtccgccaggctccagggaaggggctggagtgggtctcatccattagtcggtatagtagttacatatactacgcagactcagtgaagggccgattcaccatctccagagacaattccaagaacacgctgtatctgcaaatgaacagcctgagagccgaggacactgccgtgtattactgtgcgagagatattggcggtatggacgtctggggccaaggtacactggtcaccgtgagcagcgccagcaccaagggcccaagcgtgttccccctggcccccagcagcaagagcaccagcggcggcacagccgccctgggctgcctggtgaaggactacttccccgagcccgtgaccgtgtcctggaacagcggagccctgacctccggcgtgcacaccttccccgccgtgctgcagagcagcggcctgtacagcctgagcagcgtggtgaccgtgcccagcagcagcctgggcacccagacctacatctgtaacgtgaaccacaagcccagcaacaccaaggtggacaagaaggtggagcccaagagctgtgacaagacccacacctgccccccctgcccagcccccgagctgctgggcggacccagcgtgttcctgttcccccccaagcccaaggacaccctgatgatcagcagaacccccgaggtgacctgtgtggtggtggacgtgtcccacgaggacccagaggtgaagttcaactggtacgtggacggcgtggaggtgcacaacgccaagaccaagcccagagaggagcagtacaacagcacctacagggtggtgtccgtgctgaccgtgctgcaccaggactggctgaacggcaaggagtacaagtgtaaggtgtccaacaaggccctgccagccccaatcgaaaagaccatcagcaaggccaagggccagccaagagagccccaggtgtacaccctgccacccagcagggacgagctgaccaagaaccaggtgtccctgacctgtctggtgaagggcttctacccaagcgacatcgccgtggagtgggagagcaacggccagcccgagaacaactacaagaccacccccccagtgctggacagcgacggcagcttcttcctgtacagcaagctgaccgtggacaagagcagatggcagcagggcaacgtgttcagctgctccgtgatgcacgaggccctgcacaaccactacacccagaagagcctgagcctgtccccaggcaag

SEQ ID NO: 255 - DNA, 1338 bp, synthetic construct
  misc_feature 1..1338: note = N-HC-2
  source 1..1338: mol_type = other DNA
gaggtgcagctgttggagtctgggggaggcttggtacagcctggggggtccctgagactctcctgtgcagcctctggattcaccttcagtgactactacatgaactgggtccgccaggctccagggaaggggctggagtgggtctcatccattagtcggtatagtggctacgtttactacgcagactcagtgaagggccgattcaccatctccagagacaattccaagaacacgctgtatctgcaaatgaacagcctgagagccgaggacactgccgtgtattactgtgcgagagatattggcggtatggacgtctggggccaaggtacactggtcaccgtgagcagcgccagcaccaagggcccaagcgtgttccccctggcccccagcagcaagagcaccagcggcggcacagccgccctgggctgcctggtgaaggactacttccccgagcccgtgaccgtgtcctggaacagcggagccctgacctccggcgtgcacaccttccccgccgtgctgcagagcagcggcctgtacagcctgagcagcgtggtgaccgtgcccagcagcagcctgggcacccagacctacatctgtaacgtgaaccacaagcccagcaacaccaaggtggacaagaaggtggagcccaagagctgtgacaagacccacacctgccccccctgcccagcccccgagctgctgggcggacccagcgtgttcctgttcccccccaagcccaaggacaccctgatgatcagcagaacccccgaggtgacctgtgtggtggtggacgtgtcccacgaggacccagaggtgaagttcaactggtacgtggacggcgtggaggtgcacaacgccaagaccaagcccagagaggagcagtacaacagcacctacagggtggtgtccgtgctgaccgtgctgcaccaggactggctgaacggcaaggagtacaagtgtaaggtgtccaacaaggccctgccagccccaatcgaaaagaccatcagcaaggccaagggccagccaagagagccccaggtgtacaccctgccacccagcagggacgagctgaccaagaaccaggtgtccctgacctgtctggtgaagggcttctacccaagcgacatcgccgtggagtgggagagcaacggccagcccgagaacaactacaagaccacccccccagtgctggacagcgacggcagcttcttcctgtacagcaagctgaccgtggacaagagcagatggcagcagggcaacgtgttcagctgctccgtgatgcacgaggccctgcacaaccactacacccagaagagcctgagcctgtccccaggcaag

SEQ ID NO: 256 - DNA, 1338 bp, synthetic construct
  misc_feature 1..1338: note = N-HC-3
  source 1..1338: mol_type = other DNA
gaggtgcagctgttggagtctgggggaggcttggtacagcctggggggtccctgagactctcctgtgcagcctctggattcaccttcagtgactactacatggactgggtccgccaggctccagggaaggggctggagtgggtctcatccattagtcggtatagtggctacgtttactacgcagactcagtgaagggccgattcaccatctccagagacaattccaagaacacgctgtatctgcaaatgaacagcctgagagccgaggacactgccgtgtattactgtgcgagagatattggcggtatggacgtctggggccaaggtacactggtcaccgtgagcagcgccagcaccaagggcccaagcgtgttccccctggcccccagcagcaagagcaccagcggcggcacagccgccctgggctgcctggtgaaggactacttccccgagcccgtgaccgtgtcctggaacagcggagccctgacctccggcgtgcacaccttccccgccgtgctgcagagcagcggcctgtacagcctgagcagcgtggtgaccgtgcccagcagcagcctgggcacccagacctacatctgtaacgtgaaccacaagcccagcaacaccaaggtggacaagaaggtggagcccaagagctgtgacaagacccacacctgccccccctgcccagcccccgagctgctgggcggacccagcgtgttcctgttcccccccaagcccaaggacaccctgatgatcagcagaacccccgaggtgacctgtgtggtggtggacgtgtcccacgaggacccagaggtgaagttcaactggtacgtggacggcgtggaggtgcacaacgccaagaccaagcccagagaggagcagtacaacagcacctacagggtggtgtccgtgctgaccgtgctgcaccaggactggctgaacggcaaggagtacaagtgtaaggtgtccaacaaggccctgccagccccaatcgaaaagaccatcagcaaggccaagggccagccaagagagccccaggtgtacaccctgccacccagcagggacgagctgaccaagaaccaggtgtccctgacctgtctggtgaagggcttctacccaagcgacatcgccgtggagtgggagagcaacggccagcccgagaacaactacaagaccacccccccagtgctggacagcgacggcagcttcttcctgtacagcaagctgaccgtggacaagagcagatggcagcagggcaacgtgttcagctgctccgtgatgcacgaggccctgcacaaccactacacccagaagagcctgagcctgtccccaggcaag

SEQ ID NO: 257 - DNA, 1338 bp, synthetic construct
  misc_feature 1..1338: note = N-HC-4
  source 1..1338: mol_type = other DNA
gaggtgcagctgttggagtctgggggaggcttggtacagcctggggggtccctgagactctcctgtgcagcctctggattcaccttcagtgactactacatggactgggtccgccaggctccagggaaggggctggagtgggtctcatccattagtcgggctagtagctacgtttactacgcagactcagtgaagggccgattcaccatctccagagacaattccaagaacacgctgtatctgcaaatgaacagcctgagagccgaggacactgccgtgtattactgtgcgagagatattggcggtatggacgtctggggccaaggtacactggtcaccgtgagcagcgccagcaccaagggcccaagcgtgttccccctggcccccagcagcaagagcaccagcggcggcacagccgccctgggctgcctggtgaaggactacttccccgagcccgtgaccgtgtcctggaacagcggagccctgacctccggcgtgcacaccttccccgccgtgctgcagagcagcggcctgtacagcctgagcagcgtggtgaccgtgcccagcagcagcctgggcacccagacctacatctgtaacgtgaaccacaagcccagcaacaccaaggtggacaagaaggtggagcccaagagctgtgacaagacccacacctgccccccctgcccagcccccgagctgctgggcggacccagcgtgttcctgttcccccccaagcccaaggacaccctgatgatcagcagaacccccgaggtgacctgtgtggtggtggacgtgtcccacgaggacccagaggtgaagttcaactggtacgtggacggcgtggaggtgcacaacgccaagaccaagcccagagaggagcagtacaacagcacctacagggtggtgtccgtgctgaccgtgctgcaccaggactggctgaacggcaaggagtacaagtgtaaggtgtccaacaaggccctgccagccccaatcgaaaagaccatcagcaaggccaagggccagccaagagagccccaggtgtacaccctgccacccagcagggacgagctgaccaagaaccaggtgtccctgacctgtctggtgaagggcttctacccaagcgacatcgccgtggagtgggagagcaacggccagcccgagaacaactacaagaccacccccccagtgctggacagcgacggcagcttcttcctgtacagcaagctgaccgtggacaagagcagatggcagcagggcaacgtgttcagctgctccgtgatgcacgaggccctgcacaaccactacacccagaagagcctgagcctgtccccaggcaag

SEQ ID NO: 258 - DNA, 1338 bp, synthetic construct
  misc_feature 1..1338: note = N-HC-5
  source 1..1338: mol_type = other DNA
gaggtgcagctgttggagtctgggggaggcttggtacagcctggggggtccctgagactctcctgtgcagcctctggattcaccttcagtgactactacatgaactgggtccgccaggctccagggaaggggctggagtgggtctcatccattagtcggtatagtggctacatatactacgcagactcagtgaagggccgattcaccatctccagagacaattccaagaacacgctgtatctgcaaatgaacagcctgagagccgaggacactgccgtgtattactgtgcgagagatattggcggtatggacgtctggggccaaggtacactggtcaccgtgagcagcgccagcaccaagggcccaagcgtgttccccctggcccccagcagcaagagcaccagcggcggcacagccgccctgggctgcctggtgaaggactacttccccgagcccgtgaccgtgtcctggaacagcggagccctgacctccggcgtgcacaccttccccgccgtgctgcagagcagcggcctgtacagcctgagcagcgtggtgaccgtgcccagcagcagcctgggcacccagacctacatctgtaacgtgaaccacaagcccagcaacaccaaggtggacaagaaggtggagcccaagagctgtgacaagacccacacctgccccccctgcccagcccccgagctgctgggcggacccagcgtgttcctgttcccccccaagcccaaggacaccctgatgatcagcagaacccccgaggtgacctgtgtggtggtggacgtgtcccacgaggacccagaggtgaagttcaactggtacgtggacggcgtggaggtgcacaacgccaagaccaagcccagagaggagcagtacaacagcacctacagggtggtgtccgtgctgaccgtgctgcaccaggactggctgaacggcaaggagtacaagtgtaaggtgtccaacaaggccctgccagccccaatcgaaaagaccatcagcaaggccaagggccagccaagagagccccaggtgtacaccctgccacccagcagggacgagctgaccaagaaccaggtgtccctgacctgtctggtgaagggcttctacccaagcgacatcgccgtggagtgggagagcaacggccagcccgagaacaactacaagaccacccccccagtgctggacagcgacggcagcttcttcctgtacagcaagctgaccgtggacaagagcagatggcagcagggcaacgtgttcagctgctccgtgatgcacgaggccctgcacaaccactacacccagaagagcctgagcctgtccccaggcaag

SEQ ID NO: 259 - DNA, 1338 bp, synthetic construct
  misc_feature 1..1338: note = N-HC-6
  source 1..1338: mol_type = other DNA
gaggtgcagctgttggagtctgggggaggcttggtacagcctggggggtccctgagactctcctgtgcagcctcgggattcaccttcagtgtctactacatgaactgggtccgccaggctccagggaaggggctggagtgggtctcatccattagtcggtatagtggctacgtttactacgcagactcagtgaagggccgattcaccatctccagagacaattccaagaacacgctgtatctgcaaatgaacagcctgagagccgaggacactgccgtgtattactgtgcgagagatattggcggtatggacgtctggggccaaggtacactggtcaccgtgagcagcgccagcaccaagggcccaagcgtgttccccctggcccccagcagcaagagcaccagcggcggcacagccgccctgggctgcctggtgaaggactacttccccgagcccgtgaccgtgtcctggaacagcggagccctgacctccggcgtgcacaccttccccgccgtgctgcagagcagcggcctgtacagcctgagcagcgtggtgaccgtgcccagcagcagcctgggcacccagacctacatctgtaacgtgaaccacaagcccagcaacaccaaggtggacaagaaggtggagcccaagagctgtgacaagacccacacctgccccccctgcccagcccccgagctgctgggcggacccagcgtgttcctgttcccccccaagcccaaggacaccctgatgatcagcagaacccccgaggtgacctgtgtggtggtggacgtgtcccacgaggacccagaggtgaagttcaactggtacgtggacggcgtggaggtgcacaacgccaagaccaagcccagagaggagcagtacaacagcacctacagggtggtgtccgtgctgaccgtgctgcaccaggactggctgaacggcaaggagtacaagtgtaaggtgtccaacaaggccctgccagccccaatcgaaaagaccatcagcaaggccaagggccagccaagagagccccaggtgtacaccctgccacccagcagggacgagctgaccaagaaccaggtgtccctgacctgtctggtgaagggcttctacccaagcgacatcgccgtggagtgggagagcaacggccagcccgagaacaactacaagaccacccccccagtgctggacagcgacggcagcttcttcctgtacagcaagctgaccgtggacaagagcagatggcagcagggcaacgtgttcagctgctccgtgatgcacgaggccctgcacaaccactacacccagaagagcctgagcctgtccccaggcaag

SEQ ID NO: 260 - DNA, 1338 bp, synthetic construct
  misc_feature 1..1338: note = N-HC-7
  source 1..1338: mol_type = other DNA
gaggtgcagctgttggagtctgggggaggcttggtacagcctggggggtccctgagactctcctgtgcagcctctggattcaccttcagtgactactacgtgaactgggtccgccaggctccagggaaggggctggagtgggtctcatccattagtcggtatagtggctacgtttactacgcagactcagtgaagggccgattcaccatctccagagacaattccaagaacacgctgtatctgcaaatgaacagcctgagagccgaggacactgccgtgtattactgtgcgagagatattggcggtatggacgtctggggccaaggtacactggtcaccgtgagcagcgccagcaccaagggcccaagcgtgttccccctggcccccagcagcaagagcaccagcggcggcacagccgccctgggctgcctggtgaaggactacttccccgagcccgtgaccgtgtcctggaacagcggagccctgacctccggcgtgcacaccttccccgccgtgctgcagagcagcggcctgtacagcctgagcagcgtggtgaccgtgcccagcagcagcctgggcacccagacctacatctgtaacgtgaaccacaagcccagcaacaccaaggtggacaagaaggtggagcccaagagctgtgacaagacccacacctgccccccctgcccagcccccgagctgctgggcggacccagcgtgttcctgttcccccccaagcccaaggacaccctgatgatcagcagaacccccgaggtgacctgtgtggtggtggacgtgtcccacgaggacccagaggtgaagttcaactggtacgtggacggcgtggaggtgcacaacgccaagaccaagcccagagaggagcagtacaacagcacctacagggtggtgtccgtgctgaccgtgctgcaccaggactggctgaacggcaaggagtacaagtgtaaggtgtccaacaaggccctgccagccccaatcgaaaagaccatcagcaaggccaagggccagccaagagagccccaggtgtacaccctgccacccagcagggacgagctgaccaagaaccaggtgtccctgacctgtctggtgaagggcttctacccaagcgacatcgccgtggagtgggagagcaacggccagcccgagaacaactacaagaccacccccccagtgctggacagcgacggcagcttcttcctgtacagcaagctgaccgtggacaagagcagatggcagcagggcaacgtgttcagctgctccgtgatgcacgaggccctgcacaaccactacacccagaagagcctgagcctgtccccaggcaag

SEQ ID NO: 261 - DNA, 1347 bp, synthetic construct
  misc_feature 1..1347: note = N-HC-8
  source 1..1347: mol_type = other DNA
gaggtgcagctgttggagtctgggggaggcttggtacagcctgggggaagcttgagactctcctgtgcagcctctggattcaccttcagtaattactacatgcactgggtccgccaagctccagggaaggggctggagtgggtctcatccattagtgctaggagtcgttaccactactacgcagactcagtgaagggccgattcaccatctccagagacaattccaagaacacgctgtatctgcaaatgaacagcctgagagccgaggacactgccgtgtattactgtgcgagacttgctacgaggcataatgcttttgatatctggggccagggtacactggtcaccgtgagctcagccagcaccaagggcccaagcgtgttccccctggcccccagcagcaagagcaccagcggcggcacagccgccctgggctgcctggtgaaggactacttccccgagcccgtgaccgtgtcctggaacagcggagccctgacctccggcgtgcacaccttccccgccgtgctgcagagcagcggcctgtacagcctgagcagcgtggtgaccgtgcccagcagcagcctgggcacccagacctacatctgtaacgtgaaccacaagcccagcaacaccaaggtggacaagaaggtggagcccaagagctgtgacaagacccacacctgccccccctgcccagcccccgagctgctgggcggacccagcgtgttcctgttcccccccaagcccaaggacaccctgatgatcagcagaacccccgaggtgacctgtgtggtggtggacgtgtcccacgaggacccagaggtgaagttcaactggtacgtggacggcgtggaggtgcacaacgccaagaccaagcccagagaggagcagtacaacagcacctacagggtggtgtccgtgctgaccgtgctgcaccaggactggctgaacggcaaggagtacaagtgtaaggtgtccaacaaggccctgccagccccaatcgaaaagaccatcagcaaggccaagggccagccaagagagccccaggtgtacaccctgccacccagcagggacgagctgaccaagaaccaggtgtccctgacctgtctggtgaagggcttctacccaagcgacatcgccgtggagtgggagagcaacggccagcccgagaacaactacaagaccacccccccagtgctggacagcgacggcagcttcttcctgtacagcaagctgaccgtggacaagagcagatggcagcagggcaacgtgttcagctgctccgtgatgcacgaggccctgcacaaccactacacccagaagagcctgagcctgtccccaggcaag

SEQ ID NO: 262 - DNA, 1347 bp, synthetic construct
  misc_feature 1..1347: note = N-HC-9
  source 1..1347: mol_type = other DNA
gaggtgcagctgttggagtctgggggaggcttggtacagcctgggggaagcttgagactctcctgtgcagcatctggattcaccttcagtaattactacatgcactgggtccgccaagctccagggaaggggctggagtgggtctcatccattagtgctcgtagtagttacatatactacgcagactcagtgaagggccgattcaccatctccagagacaattccaagaacacgctgtatctgcaaatgaacagcctgagagccgaggacactgccgtgtattactgtgcgagacttgctacgaggaataatgcttttgatatctggggccagggtacactggtcaccgtgagctcagccagcaccaagggcccaagcgtgttccccctggcccccagcagcaagagcaccagcggcggcacagccgccctgggctgcctggtgaaggactacttccccgagcccgtgaccgtgtcctggaacagcggagccctgacctccggcgtgcacaccttccccgccgtgctgcagagcagcggcctgtacagcctgagcagcgtggtgaccgtgcccagcagcagcctgggcacccagacctacatctgtaacgtgaaccacaagcccagcaacaccaaggtggacaagaaggtggagcccaagagctgtgacaagacccacacctgccccccctgcccagcccccgagctgctgggcggacccagcgtgttcctgttcccccccaagcccaaggacaccctgatgatcagcagaacccccgaggtgacctgtgtggtggtggacgtgtcccacgaggacccagaggtgaagttcaactggtacgtggacggcgtggaggtgcacaacgccaagaccaagcccagagaggagcagtacaacagcacctacagggtggtgtccgtgctgaccgtgctgcaccaggactggctgaacggcaaggagtacaagtgtaaggtgtccaacaaggccctgccagccccaatcgaaaagaccatcagcaaggccaagggccagccaagagagccccaggtgtacaccctgccacccagcagggacgagctgaccaagaaccaggtgtccctgacctgtctggtgaagggcttctacccaagcgacatcgccgtggagtgggagagcaacggccagcccgagaacaactacaagaccacccccccagtgctggacagcgacggcagcttcttcctgtacagcaagctgaccgtggacaagagcagatggcagcagggcaacgtgttcagctgctccgtgatgcacgaggccctgcacaaccactacacccagaagagcctgagcctgtccccaggcaag

SEQ ID NO: 263 - DNA, 1347 bp, synthetic construct
  misc_feature 1..1347: note = N-HC-10
  source 1..1347: mol_type = other DNA
gaggtgcagctgttggagtctgggggaggcttggtacaacctgggggaagcttgagactctcctgtgcagcctctggattcaccttcagtcattactacatgcactgggtccgccaagctccagggaaggggctggagtgggtctcatccattagtgctcttagtagttacatatactacgcagactcagtgaggggccgattcaccatctccagagacaattccaagaacacgctgtatctgcaaatgaacagcctgagagccgaggacactgccgtgtattactgtgcgagacttgctacgaggcgtgatgcttttgatatctggggccagggtacactggtcaccgtgagctcagccagcaccaagggcccaagcgtgttccccctggcccccagcagcaagagcaccagcggcggcacagccgccctgggctgcctggtgaaggactacttccccgagcccgtgaccgtgtcctggaacagcggagccctgacctccggcgtgcacaccttccccgccgtgctgcagagcagcggcctgtacagcctgagcagcgtggtgaccgtgcccagcagcagcctgggcacccagacctacatctgtaacgtgaaccacaagcccagcaacaccaaggtggacaagaaggtggagcccaagagctgtgacaagacccacacctgccccccctgcccagcccccgagctgctgggcggacccagcgtgttcctgttcccccccaagcccaaggacaccctgatgatcagcagaacccccgaggtgacctgtgtggtggtggacgtgtcccacgaggacccagaggtgaagttcaactggtacgtggacggcgtggaggtgcacaacgccaagaccaagcccagagaggagcagtacaacagcacctacagggtggtgtccgtgctgaccgtgctgcaccaggactggctgaacggcaaggagtacaagtgtaaggtgtccaacaaggccctgccagccccaatcgaaaagaccatcagcaaggccaagggccagccaagagagccccaggtgtacaccctgccacccagcagggacgagctgaccaagaaccaggtgtccctgacctgtctggtgaagggcttctacccaagcgacatcgccgtggagtgggagagcaacggccagcccgagaacaactacaagaccacccccccagtgctggacagcgacggcagcttcttcctgtacagcaagctgaccgtggacaagagcagatggcagcagggcaacgtgttcagctgctccgtgatgcacgaggccctgcacaaccactacacccagaagagcctgagcctgtccccaggcaag

SEQ ID NO: 264 - DNA, 1347 bp, synthetic construct
  misc_feature 1..1347: note = N-HC-11
  source 1..1347: mol_type = other DNA
gaggtgcagctgttggagtctgggggaggcttggtacagcctgggggaagcttgagactctcctgtgcagcctctggattcaccttcagtcgttactacatgcactgggtccgccaagctccagggaaggggctggagtgggtctcatccattagtgctcagagtagtcacatatactacgcagactcagtggagggccgattcaccatctccagagacaattccaagaacacgctgtatctgcaaatgaacagcctgagagccgaggacactgccgtgtattactgtgcgagacttgctacgaggcaaaacgcttttgatatctggggccagggtacactggtcaccgtgagctcagccagcaccaagggcccaagcgtgttccccctggcccccagcagcaagagcaccagcggcggcacagccgccctgggctgcctggtgaaggactacttccccgagcccgtgaccgtgtcctggaacagcggagccctgacctccggcgtgcacaccttccccgccgtgctgcagagcagcggcctgtacagcctgagcagcgtggtgaccgtgcccagcagcagcctgggcacccagacctacatctgtaacgtgaaccacaagcccagcaacaccaaggtggacaagaaggtggagcccaagagctgtgacaagacccacacctgccccccctgcccagcccccgagctgctgggcggacccagcgtgttcctgttcccccccaagcccaaggacaccctgatgatcagcagaacccccgaggtgacctgtgtggtggtggacgtgtcccacgaggacccagaggtgaagttcaactggtacgtggacggcgtggaggtgcacaacgccaagaccaagcccagagaggagcagtacaacagcacctacagggtggtgtccgtgctgaccgtgctgcaccaggactggctgaacggcaaggagtacaagtgtaaggtgtccaacaaggccctgccagccccaatcgaaaagaccatcagcaaggccaagggccagccaagagagccccaggtgtacaccctgccacccagcagggacgagctgaccaagaaccaggtgtccctgacctgtctggtgaagggcttctacccaagcgacatcgccgtggagtgggagagcaacggccagcccgagaacaactacaagaccacccccccagtgctggacagcgacggcagcttcttcctgtacagcaagctgaccgtggacaagagcagatggcagcagggcaacgtgttcagctgctccgtgatgcacgaggccctgcacaaccactacacccagaagagcctgagcctgtccccaggcaag

SEQ ID NO: 265 - DNA, 1347 bp, synthetic construct
  misc_feature 1..1347: note = N-HC-12
  source 1..1347: mol_type = other DNA
gaggtgcagctgttggagtctgggggaggcttggtacagcctgggggaagcttgagactctcctgtgcagcctctggattcaccttcagtaattactacatgcactgggtccgccaagctccagggaaggggctggagtgggtctcatccattagtgctcggagtagctacctatactacgcagactcagtgaagggccgattcaccatctccagagacaattccaagaacacgctgtatctgcaaatgaacagcctgagagccgaggacactgccgtgtattactgtgcgagacttgctaccaggcatgtcgcttttgatatctggggccagggtacactggtcaccgtgagctcagccagcaccaagggcccaagcgtgttccccctggcccccagcagcaagagcaccagcggcggcacagccgccctgggctgcctggtgaaggactacttccccgagcccgtgaccgtgtcctggaacagcggagccctgacctccggcgtgcacaccttccccgccgtgctgcagagcagcggcctgtacagcctgagcagcgtggtgaccgtgcccagcagcagcctgggcacccagacctacatctgtaacgtgaaccacaagcccagcaacaccaaggtggacaagaaggtggagcccaagagctgtgacaagacccacacctgccccccctgcccagcccccgagctgctgggcggacccagcgtgttcctgttcccccccaagcccaaggacaccctgatgatcagcagaacccccgaggtgacctgtgtggtggtggacgtgtcccacgaggacccagaggtgaagttcaactggtacgtggacggcgtggaggtgcacaacgccaagaccaagcccagagaggagcagtacaacagcacctacagggtggtgtccgtgctgaccgtgctgcaccaggactggctgaacggcaaggagtacaagtgtaaggtgtccaacaaggccctgccagccccaatcgaaaagaccatcagcaaggccaagggccagccaagagagccccaggtgtacaccctgccacccagcagggacgagctgaccaagaaccaggtgtccctgacctgtctggtgaagggcttctacccaagcgacatcgccgtggagtgggagagcaacggccagcccgagaacaactacaagaccacccccccagtgctggacagcgacggcagcttcttcctgtacagcaagctgaccgtggacaagagcagatggcagcagggcaacgtgttcagctgctccgtgatgcacgaggccctgcacaaccactacacccagaagagcctgagcctgtccccaggcaag

SEQ ID NO: 266 - DNA, 1347 bp, synthetic construct
  misc_feature 1..1347: note = N-HC-13
  source 1..1347: mol_type = other DNA
gaggtgcagctgttggagtctgggggaggcttggtacagcctgggggaagcttgagactctcctgtgcagcctctggattcaccttcagtaattactacatgcactgggtccgccaagctccagggaaggggctggagtgggtctcatccattagtgctcggagtagctacatatactacgcagactcagtgaagggccgattcaccatctccagagacaattccaagaacacgctgtatctgcaaatgaacagcctgagagccgaggacactgccgtgtattactgtgcgagacttgctaccaggcatggcgcttttgatatctggggccagggtacactggtcaccgtgagctcagccagcaccaagggcccaagcgtgttccccctggcccccagcagcaagagcaccagcggcggcacagccgccctgggctgcctggtgaaggactacttccccgagcccgtgaccgtgtcctggaacagcggagccctgacctccggcgtgcacaccttccccgccgtgctgcagagcagcggcctgtacagcctgagcagcgtggtgaccgtgcccagcagcagcctgggcacccagacctacatctgtaacgtgaaccacaagcccagcaacaccaaggtggacaagaaggtggagcccaagagctgtgacaagacccacacctgccccccctgcccagcccccgagctgctgggcggacccagcgtgttcctgttcccccccaagcccaaggacaccctgatgatcagcagaacccccgaggtgacctgtgtggtggtggacgtgtcccacgaggacccagaggtgaagttcaactggtacgtggacggcgtggaggtgcacaacgccaagaccaagcccagagaggagcagtacaacagcacctacagggtggtgtccgtgctgaccgtgctgcaccaggactggctgaacggcaaggagtacaagtgtaaggtgtccaacaaggccctgccagccccaatcgaaaagaccatcagcaaggccaagggccagccaagagagccccaggtgtacaccctgccacccagcagggacgagctgaccaagaaccaggtgtccctgacctgtctggtgaagggcttctacccaagcgacatcgccgtggagtgggagagcaacggccagcccgagaacaactacaagaccacccccccagtgctggacagcgacggcagcttcttcctgtacagcaagctgaccgtggacaagagcagatggcagcagggcaacgtgttcagctgctccgtgatgcacgaggccctgcacaaccactacacccagaagagcctgagcctgtccccaggcaag

SEQ ID NO: 267 - DNA, 1347 bp, synthetic construct
  misc_feature 1..1347: note = N-HC-14
  source 1..1347: mol_type = other DNA
gaggtgcagctgttggagtctgggggaggcttggtacagcctgggggaagcttgagactctcctgtgcagcctctggattcaccttcagtaattactacatgcactgggtccgccaagctccagggaaggggctggagtgggtctcatccattagtgctcggagtagctacatatactacgcagactcagtgaagggccgattcaccatctccagagacaattccaagaacacgctgtatctgcaaatgaacagcctgagagccgaggacactgccgtgtattactgtgcgagacttgctaccaggcataacgcttttgatatctggggccagggtacactggtcaccgtgagctcagccagcaccaagggcccaagcgtgttccccctggcccccagcagcaagagcaccagcggcggcacagccgccctgggctgcctggtgaaggactacttccccgagcccgtgaccgtgtcctggaacagcggagccctgacctccggcgtgcacaccttccccgccgtgctgcagagcagcggcctgtacagcctgagcagcgtggtgaccgtgcccagcagcagcctgggcacccagacctacatctgtaacgtgaaccacaagcccagcaacaccaaggtggacaagaaggtggagcccaagagctgtgacaagacccacacctgccccccctgcccagcccccgagctgctgggcggacccagcgtgttcctgttcccccccaagcccaaggacaccctgatgatcagcagaacccccgaggtgacctgtgtggtggtggacgtgtcccacgaggacccagaggtgaagttcaactggtacgtggacggcgtggaggtgcacaacgccaagaccaagcccagagaggagcagtacaacagcacctacagggtggtgtccgtgctgaccgtgctgcaccaggactggctgaacggcaaggagtacaagtgtaaggtgtccaacaaggccctgccagccccaatcgaaaagaccatcagcaaggccaagggccagccaagagagccccaggtgtacaccctgccacccagcagggacgagctgaccaagaaccaggtgtccctgacctgtctggtgaagggcttctacccaagcgacatcgccgtggagtgggagagcaacggccagcccgagaacaactacaagaccacccccccagtgctggacagcgacggcagcttcttcctgtacagcaagctgaccgtggacaagagcagatggcagcagggcaacgtgttcagctgctccgtgatgcacgaggccctgcacaaccactacacccagaagagcctgagcctgtccccaggcaag

SEQ ID NO: 268 - DNA, 1347 bp, synthetic construct
  misc_feature 1..1347: note = N-HC-15
  source 1..1347: mol_type = other DNA
gaggtgcagctgttggagtctgggggaggcttggtacagcctgggggaagcttgagactctcctgtgcagcctctggattcaccttcagtaattactacatgcactgggtccgccaagctccagggaaggggctggagtgggtctcatccattagtgctcgcagtagctaccgctactacgcagactcagtgaagggccgattcaccatctccagagacaattccaagaacacgctgtatctgcaaatgaacagcctgagagccgaggacactgccgtgtattactgtgcgagacttgctaccaggcatctcgcttttgatatctggggccagggtacactggtcaccgtgagctcagccagcaccaagggcccaagcgtgttccccctggcccccagcagcaagagcaccagcggcggcacagccgccctgggctgcctggtgaaggactacttccccgagcccgtgaccgtgtcctggaacagcggagccctgacctccggcgtgcacaccttccccgccgtgctgcagagcagcggcctgtacagcctgagcagcgtggtgaccgtgcccagcagcagcctgggcacccagacctacatctgtaacgtgaaccacaagcccagcaacaccaaggtggacaagaaggtggagcccaagagctgtgacaagacccacacctgccccccctgcccagcccccgagctgctgggcggacccagcgtgttcctgttcccccccaagcccaaggacaccctgatgatcagcagaacccccgaggtgacctgtgtggtggtggacgtgtcccacgaggacccagaggtgaagttcaactggtacgtggacggcgtggaggtgcacaacgccaagaccaagcccagagaggagcagtacaacagcacctacagggtggtgtccgtgctgaccgtgctgcaccaggactggctgaacggcaaggagtacaagtgtaaggtgtccaacaaggccctgccagccccaatcgaaaagaccatcagcaaggccaagggccagccaagagagccccaggtgtacaccctgccacccagcagggacgagctgaccaagaaccaggtgtccctgacctgtctggtgaagggcttctacccaagcgacatcgccgtggagtgggagagcaacggccagcccgagaacaactacaagaccacccccccagtgctggacagcgacggcagcttcttcctgtacagcaagctgaccgtggacaagagcagatggcagcagggcaacgtgttcagctgctccgtgatgcacgaggccctgcacaaccactacacccagaagagcctgagcctgtccccaggcaag

SEQ ID NO: 269 - DNA, 1347 bp, synthetic construct
  misc_feature 1..1347: note = N-HC-16
  source 1..1347: mol_type = other DNA
gaggtgcagctgttggagtctgggggaggcttggtacagcctgggggaagcttgagactctcctgtgcagcctctggattcaccttcagtaattactacatgcactgggtccgccaagctccagggaaggggctggagtgggtctcatccattagtgctcggagtagctacatatactacgcagactcagtgaagggccgattcaccatctccagagacaattccaagaacacgctgtatctgcaaatgaacagcctgagagccgaggacactgccgtgtattactgtgcgagacttgctaccaggcatagcgcttttgatatctggggccagggtacactggtcaccgtgagctcagccagcaccaagggcccaagcgtgttccccctggcccccagcagcaagagcaccagcggcggcacagccgccctgggctgcctggtgaaggactacttccccgagcccgtgaccgtgtcctggaacagcggagccctgacctccggcgtgcacaccttccccgccgtgctgcagagcagcggcctgtacagcctgagcagcgtggtgaccgtgcccagcagcagcctgggcacccagacctacatctgtaacgtgaaccacaagcccagcaacaccaaggtggacaagaaggtggagcccaagagctgtgacaagacccacacctgccccccctgcccagcccccgagctgctgggcggacccagcgtgttcctgttcccccccaagcccaaggacaccctgatgatcagcagaacccccgaggtgacctgtgtggtggtggacgtgtcccacgaggacccagaggtgaagttcaactggtacgtggacggcgtggaggtgcacaacgccaagaccaagcccagagaggagcagtacaacagcacctacagggtggtgtccgtgctgaccgtgctgcaccaggactggctgaacggcaaggagtacaagtgtaaggtgtccaacaaggccctgccagccccaatcgaaaagaccatcagcaaggccaagggccagccaagagagccccaggtgtacaccctgccacccagcagggacgagctgaccaagaaccaggtgtccctgacctgtctggtgaagggcttctacccaagcgacatcgccgtggagtgggagagcaacggccagcccgagaacaactacaagaccacccccccagtgctggacagcgacggcagcttcttcctgtacagcaagctgaccgtggacaagagcagatggcagcagggcaacgtgttcagctgctccgtgatgcacgaggccctgcacaaccactacacccagaagagcctgagcctgtccccaggcaag

SEQ ID NO: 270 - DNA, 1347 bp, synthetic construct
  misc_feature 1..1347: note = N-HC-17
  source 1..1347: mol_type = other DNA
gaggtgcagctgttggagtctgggggaggcttggtacagcctgggggaagcttgagactctcctgtgcagcctctggattcaccttcagtcgctactacatgcactgggtccgccaagctccagggaaggggctggagtgggtctcatccattagtgctcggagtagctacatctactacgcagattcagtgaagggccgattcaccatctccagagacaattccaagaacacgctgtatctgcaaatgaacagcctgagagccgaggacactgccgtgtattactgtgcgagacttgctaccaggcgcgacgcttttgatatctggggccagggtacactggtcaccgtgagctcagccagcaccaagggcccaagcgtgttccccctggcccccagcagcaagagcaccagcggcggcacagccgccctgggctgcctggtgaaggactacttccccgagcccgtgaccgtgtcctggaacagcggagccctgacctccggcgtgcacaccttccccgccgtgctgcagagcagcggcctgtacagcctgagcagcgtggtgaccgtgcccagcagcagcctgggcacccagacctacatctgtaacgtgaaccacaagcccagcaacaccaaggtggacaagaaggtggagcccaagagctgtgacaagacccacacctgccccccctgcccagcccccgagctgctgggcggacccagcgtgttcctgttcccccccaagcccaaggacaccctgatgatcagcagaacccccgaggtgacctgtgtggtggtggacgtgtcccacgaggacccagaggtgaagttcaactggtacgtggacggcgtggaggtgcacaacgccaagaccaagcccagagaggagcagtacaacagcacctacagggtggtgtccgtgctgaccgtgctgcaccaggactggctgaacggcaaggagtacaagtgtaaggtgtccaacaaggccctgccagccccaatcgaaaagaccatcagcaaggccaagggccagccaagagagccccaggtgtacaccctgccacccagcagggacgagctgaccaagaaccaggtgtccctgacctgtctggtgaagggcttctacccaagcgacatcgccgtggagtgggagagcaacggccagcccgagaacaactacaagaccacccccccagtgctggacagcgacggcagcttcttcctgtacagcaagctgaccgtggacaagagcagatggcagcagggcaacgtgttcagctgctccgtgatgcacgaggccctgcacaaccactacacccagaagagcctgagcctgtccccaggcaag

SEQ ID NO: 271 - DNA, 1347 bp, synthetic construct
  misc_feature 1..1347: note = N-HC-18
  source 1..1347: mol_type = other DNA
gaggtgcagctgttggagtctgggggaggcttggtacagcctgggggaagcttgagactctcctgtgcagcctctggattcaccttcagtaactactacatgcactgggtccgccaagctccagggaaggggctggagtgggtctcatccattagtgctcggagtagctaccgctactacgcagattcagtgaagggccgattcaccatctccagagacaattccaagaacacgctgtatctgcaaatgaacagcctgagagccgaggacactgccgtgtattactgtgcgagacttgctaccaggcacagcgcttttgatatctggggccagggtacactggtcaccgtgagctcagccagcaccaagggcccaagcgtgttccccctggcccccagcagcaagagcaccagcggcggcacagccgccctgggctgcctggtgaaggactacttccccgagcccgtgaccgtgtcctggaacagcggagccctgacctccggcgtgcacaccttccccgccgtgctgcagagcagcggcctgtacagcctgagcagcgtggtgaccgtgcccagcagcagcctgggcacccagacctacatctgtaacgtgaaccacaagcccagcaacaccaaggtggacaagaaggtggagcccaagagctgtgacaagacccacacctgccccccctgcccagcccccgagctgctgggcggacccagcgtgttcctgttcccccccaagcccaaggacaccctgatgatcagcagaacccccgaggtgacctgtgtggtggtggacgtgtcccacgaggacccagaggtgaagttcaactggtacgtggacggcgtggaggtgcacaacgccaagaccaagcccagagaggagcagtacaacagcacctacagggtggtgtccgtgctgaccgtgctgcaccaggactggctgaacggcaaggagtacaagtgtaaggtgtccaacaaggccctgccagccccaatcgaaaagaccatcagcaaggccaagggccagccaagagagccccaggtgtacaccctgccacccagcagggacgagctgaccaagaaccaggtgtccctgacctgtctggtgaagggcttctacccaagcgacatcgccgtggagtgggagagcaacggccagcccgagaacaactacaagaccacccccccagtgctggacagcgacggcagcttcttcctgtacagcaagctgaccgtggacaagagcagatggcagcagggcaacgtgttcagctgctccgtgatgcacgaggccctgcacaaccactacacccagaagagcctgagcctgtccccaggcaag

SEQ ID NO: 272 - DNA, 1347 bp, synthetic construct
  misc_feature 1..1347: note = N-HC-19
  source 1..1347: mol_type = other DNA
gaggtgcagctgttggagtctgggggaggcttggtacagcctgggggaagcttgagactctcctgtgcagcctctggattcaccttcagtaactactacatgcactgggtccgccaagctccagggaaggggctggagtgggtctcatccattagtgctcggagtagctacatctactacgcaggttcagtgaagggccgattcaccatctccagagacaattccaagaacacgctgtatctgcaaatgaacagcctgagagccgaggacactgccgtgtattactgtgcgagacttggtaccaggcgcgtcgcttttgatatctggggccagggtacactggtcaccgtgagctcagccagcaccaagggcccaagcgtgttccccctggcccccagcagcaagagcaccagcggcggcacagccgccctgggctgcctggtgaaggactacttccccgagcccgtgaccgtgtcctggaacagcggagccctgacctccggcgtgcacaccttccccgccgtgctgcagagcagcggcctgtacagcctgagcagcgtggtgaccgtgcccagcagcagcctgggcacccagacctacatctgtaacgtgaaccacaagcccagcaacaccaaggtggacaagaaggtggagcccaagagctgtgacaagacccacacctgccccccctgcccagcccccgagctgctgggcggacccagcgtgttcctgttcccccccaagcccaaggacaccctgatgatcagcagaacccccgaggtgacctgtgtggtggtggacgtgtcccacgaggacccagaggtgaagttcaactggtacgtggacggcgtggaggtgcacaacgccaagaccaagcccagagaggagcagtacaacagcacctacagggtggtgtccgtgctgaccgtgctgcaccaggactggctgaacggcaaggagtacaagtgtaaggtgtccaacaaggccctgccagccccaatcgaaaagaccatcagcaaggccaagggccagccaagagagccccaggtgtacaccctgccacccagcagggacgagctgaccaagaaccaggtgtccctgacctgtctggtgaagggcttctacccaagcgacatcgccgtggagtgggagagcaacggccagcccgagaacaactacaagaccacccccccagtgctggacagcgacggcagcttcttcctgtacagcaagctgaccgtggacaagagcagatggcagcagggcaacgtgttcagctgctccgtgatgcacgaggccctgcacaaccactacacccagaagagcctgagcctgtccccaggcaag

SEQ ID NO: 273 - DNA, 1347 bp, synthetic construct
  misc_feature 1..1347: note = N-HC-20
  source 1..1347: mol_type = other DNA
gaggtgcagctgttggagtctgggggaggcttggtacagcctgggggaagcttgagactctcctgtgcagcctctggattcaccttcagtaactactacatgcactgggtccgccaagctccagggaaggggctggagtgggtctcatccattagttctaggagtagccaccaatactacgcaggttcagtgaagggccgattcaccatctccagagacaattccaagaacacgctgtatctgcaaatgaacagcctgagagccgaggacactgccgtgtattactgtgcgagacttggtctcaggcacgacgcttttgatatctggggccagggtacactggtcaccgtgagctcagccagcaccaagggcccaagcgtgttccccctggcccccagcagcaagagcaccagcggcggcacagccgccctgggctgcctggtgaaggactacttccccgagcccgtgaccgtgtcctggaacagcggagccctgacctccggcgtgcacaccttccccgccgtgctgcagagcagcggcctgtacagcctgagcagcgtggtgaccgtgcccagcagcagcctgggcacccagacctacatctgtaacgtgaaccacaagcccagcaacaccaaggtggacaagaaggtggagcccaagagctgtgacaagacccacacctgccccccctgcccagcccccgagctgctgggcggacccagcgtgttcctgttcccccccaagcccaaggacaccctgatgatcagcagaacccccgaggtgacctgtgtggtggtggacgtgtcccacgaggacccagaggtgaagttcaactggtacgtggacggcgtggaggtgcacaacgccaagaccaagcccagagaggagcagtacaacagcacctacagggtggtgtccgtgctgaccgtgctgcaccaggactggctgaacggcaaggagtacaagtgtaaggtgtccaacaaggccctgccagccccaatcgaaaagaccatcagcaaggccaagggccagccaagagagccccaggtgtacaccctgccacccagcagggacgagctgaccaagaaccaggtgtccctgacctgtctggtgaagggcttctacccaagcgacatcgccgtggagtgggagagcaacggccagcccgagaacaactacaagaccacccccccagtgctggacagcgacggcagcttcttcctgtacagcaagctgaccgtggacaagagcagatggcagcagggcaacgtgttcagctgctccgtgatgcacgaggccctgcacaaccactacacccagaagagcctgagcctgtccccaggcaag

SEQ ID NO: 274 - DNA, 1347 bp, synthetic construct
  misc_feature 1..1347: note = N-HC-21
  source 1..1347: mol_type = other DNA
gaggtgcagctgttggagtctgggggaggcttggtacagcctgggggaagcttgagactctcctgtgcagcctctggattcaccttcagtagctactacatgcactgggtccgccaagctccagggaaggggctggagtgggtctcatccattagtgctaggagtagctacatctactacgcagattcagtgaagggccgattcaccatctccagagacaattccaagaacacgctgtatctgcaaatgaacagcctgagagccgaggacactgccgtgtattactgtgcgagacttgctaccaggcgcatcgcttttgatatctggggccagggtacactggtcaccgtgagctcagccagcaccaagggcccaagcgtgttccccctggcccccagcagcaagagcaccagcggcggcacagccgccctgggctgcctggtgaaggactacttccccgagcccgtgaccgtgtcctggaacagcggagccctgacctccggcgtgcacaccttccccgccgtgctgcagagcagcggcctgtacagcctgagcagcgtggtgaccgtgcccagcagcagcctgggcacccagacctacatctgtaacgtgaaccacaagcccagcaacaccaaggtggacaagaaggtggagcccaagagctgtgacaagacccacacctgccccccctgcccagcccccgagctgctgggcggacccagcgtgttcctgttcccccccaagcccaaggacaccctgatgatcagcagaacccccgaggtgacctgtgtggtggtggacgtgtcccacgaggacccagaggtgaagttcaactggtacgtggacggcgtggaggtgcacaacgccaagaccaagcccagagaggagcagtacaacagcacctacagggtggtgtccgtgctgaccgtgctgcaccaggactggctgaacggcaaggagtacaagtgtaaggtgtccaacaaggccctgccagccccaatcgaaaagaccatcagcaaggccaagggccagccaagagagccccaggtgtacaccctgccacccagcagggacgagctgaccaagaaccaggtgtccctgacctgtctggtgaagggcttctacccaagcgacatcgccgtggagtgggagagcaacggccagcccgagaacaactacaagaccacccccccagtgctggacagcgacggcagcttcttcctgtacagcaagctgaccgtggacaagagcagatggcagcagggcaacgtgttcagctgctccgtgatgcacgaggccctgcacaaccactacacccagaagagcctgagcctgtccccaggcaag

SEQ ID NO: 275 - DNA, 1347 bp, synthetic construct
  misc_feature 1..1347: note = N-HC-22
  source 1..1347: mol_type = other DNA
gaggtgcagctgttggagtctgggggaggcttggtacagcctgggggaagcttgagactctcctgtgcagcctctggattcaccttcagtaattactacatgcactgggtccgccaagctccagggaaggggctggagtgggtctcatccattagtgctctgagtagctaccgatactacgcagattcagtgaagggccgattcaccatctccagagacaattccaagaacacgctgtatctgcaaatgaacagcctgagagccgaggacactgccgtgtattactgtgcgagacttgctaccaggcgcgtcgcttttgatatctggggccagggtacactggtcaccgtgagctcagccagcaccaagggcccaagcgtgttccccctggcccccagcagcaagagcaccagcggcggcacagccgccctgggctgcctggtgaaggactacttccccgagcccgtgaccgtgtcctggaacagcggagccctgacctccggcgtgcacaccttccccgccgtgctgcagagcagcggcctgtacagcctgagcagcgtggtgaccgtgcccagcagcagcctgggcacccagacctacatctgtaacgtgaaccacaagcccagcaacaccaaggtggacaagaaggtggagcccaagagctgtgacaagacccacacctgccccccctgcccagcccccgagctgctgggcggacccagcgtgttcctgttcccccccaagcccaaggacaccctgatgatcagcagaacccccgaggtgacctgtgtggtggtggacgtgtcccacgaggacccagaggtgaagttcaactggtacgtggacggcgtggaggtgcacaacgccaagaccaagcccagagaggagcagtacaacagcacctacagggtggtgtccgtgctgaccgtgctgcaccaggactggctgaacggcaaggagtacaagtgtaaggtgtccaacaaggccctgccagccccaatcgaaaagaccatcagcaaggccaagggccagccaagagagccccaggtgtacaccctgccacccagcagggacgagctgaccaagaaccaggtgtccctgacctgtctggtgaagggcttctacccaagcgacatcgccgtggagtgggagagcaacggccagcccgagaacaactacaagaccacccccccagtgctggacagcgacggcagcttcttcctgtacagcaagctgaccgtggacaagagcagatggcagcagggcaacgtgttcagctgctccgtgatgcacgaggccctgcacaaccactacacccagaagagcctgagcctgtccccaggcaag

SEQ ID NO: 276 - DNA, 1338 bp, synthetic construct
  misc_feature 1..1338: note = N-HC-23
  source 1..1338: mol_type = other DNA
gaggtgcagctgttggagtctgggggaggcttggtacagcctggggggtccctgagactctcctgtgcagcctctggattcaccttcagtgactactacatgaactgggtccgccaggctccagggaaggggctggagtgggtctcatccattagtagtagtagtagttacatatactacgcagactcagtgaagggccgattcaccatctccagagacaattccaagaacacgctgtatctgcaaatgaacagcctgagagccgaggacactgccgtgtattactgtgcgagagatattggcggtatggacgtctggggccaaggtacactggtcaccgtgagcagcgccagcaccaagggcccaagcgtgttccccctggcccccagcagcaagagcaccagcggcggcacagccgccctgggctgcctggtgaaggactacttccccgagcccgtgaccgtgtcctggaacagcggagccctgacctccggcgtgcacaccttccccgccgtgctgcagagcagcggcctgtacagcctgagcagcgtggtgaccgtgcccagcagcagcctgggcacccagacctacatctgtaacgtgaaccacaagcccagcaacaccaaggtggacaagaaggtggagcccaagagctgtgacaagacccacacctgccccccctgcccagcccccgagctgctgggcggacccagcgtgttcctgttcccccccaagcccaaggacaccctgatgatcagcagaacccccgaggtgacctgtgtggtggtggacgtgtcccacgaggacccagaggtgaagttcaactggtacgtggacggcgtggaggtgcacaacgccaagaccaagcccagagaggagcagtacaacagcacctacagggtggtgtccgtgctgaccgtgctgcaccaggactggctgaacggcaaggagtacaagtgtaaggtgtccaacaaggccctgccagccccaatcgaaaagaccatcagcaaggccaagggccagccaagagagccccaggtgtacaccctgccacccagcagggacgagctgaccaagaaccaggtgtccctgacctgtctggtgaagggcttctacccaagcgacatcgccgtggagtgggagagcaacggccagcccgagaacaactacaagaccacccccccagtgctggacagcgacggcagcttcttcctgtacagcaagctgaccgtggacaagagcagatggcagcagggcaacgtgttcagctgctccgtgatgcacgaggccctgcacaaccactacacccagaagagcctgagcctgtccccaggcaag

SEQ ID NO: 277 - DNA, 1347 bp, synthetic construct
  misc_feature 1..1347: note = N-HC-24
  source 1..1347: mol_type = other DNA
gaggtgcagctgttggagtctgggggaggcttggtacagcctgggggaagcttgagactctcctgtgcagcctctggattcaccttcagtaattactacatgcactgggtccgccaagctccagggaaggggctggagtgggtctcatccattagtagtagtagtagttacatatactacgcagactcagtgaagggccgattcaccatctccagagacaattccaagaacacgctgtatctgcaaatgaacagcctgagagccgaggacactgccgtgtattactgtgcgagacttggtacgaggcatgatgcttttgatatctggggccagggtacactggtcaccgtgagctcagccagcaccaagggcccaagcgtgttccccctggcccccagcagcaagagcaccagcggcggcacagccgccctgggctgcctggtgaaggactacttccccgagcccgtgaccgtgtcctggaacagcggagccctgacctccggcgtgcacaccttccccgccgtgctgcagagcagcggcctgtacagcctgagcagcgtggtgaccgtgcccagcagcagcctgggcacccagacctacatctgtaacgtgaaccacaagcccagcaacaccaaggtggacaagaaggtggagcccaagagctgtgacaagacccacacctgccccccctgcccagcccccgagctgctgggcggacccagcgtgttcctgttcccccccaagcccaaggacaccctgatgatcagcagaacccccgaggtgacctgtgtggtggtggacgtgtcccacgaggacccagaggtgaagttcaactggtacgtggacggcgtggaggtgcacaacgccaagaccaagcccagagaggagcagtacaacagcacctacagggtggtgtccgtgctgaccgtgctgcaccaggactggctgaacggcaaggagtacaagtgtaaggtgtccaacaaggccctgccagccccaatcgaaaagaccatcagcaaggccaagggccagccaagagagccccaggtgtacaccctgccacccagcagggacgagctgaccaagaaccaggtgtccctgacctgtctggtgaagggcttctacccaagcgacatcgccgtggagtgggagagcaacggccagcccgagaacaactacaagaccacccccccagtgctggacagcgacggcagcttcttcctgtacagcaagctgaccgtggacaagagcagatggcagcagggcaacgtgttcagctgctccgtgatgcacgaggccctgcacaaccactacacccagaagagcctgagcctgtccccaggcaag

SEQ ID NO: 278 - protein, 95 aa, Homo sapiens
DIQMTQSPSTLSASVGDRVTITCRASQSISSWLAWYQQKPGKAPKLLIYDASSLESGVPSRFSGSGSGTEFTLTISSLQPDDFATYYCQQYNSYS

SEQ ID NO: 279 - protein, 95 aa, Homo sapiens
AIQMTQSPSSLSASVGDRVTITCRASQGIRNDLGWYQQKPGKAPKLLIYAASSLQSGVPSRFSGSGSGTDFTLTISSLQPEDFATYYCLQDYNYP

SEQ ID NO: 280 - protein, 95 aa, Homo sapiens
AIRMTQSPSSFSASTGDRVTITCRASQGISSYLAWYQQKPGKAPKLLIYAASTLQSGVPSRFSGSGSGTDFTLTISCLQSEDFATYYCQQYYSYP

SEQ ID NO: 281 - protein, 95 aa, Homo sapiens
DIQLTQSPSFLSASVGDRVTITCRASQGISSYLAWYQQKPGKAPKLLIYAASTLQSGVPSRFSGSGSGTEFTLTISSLQPEDFATYYCQQLNSYP

SEQ ID NO: 282 - protein, 95 aa, Homo sapiens
DIQMTQSPSSVSASVGDRVTITCRASQGISSWLAWYQQKPGKAPKLLIYAASSLQSGVPSRFSGSGSGTDFTLTISSLQPEDFATYYCQQANSFP

SEQ ID NO: 283 - protein, 95 aa, Homo sapiens
DIQMTQSPSSLSASVGDRVTITCRASQGISNYLAWFQQKPGKAPKSLIYAASSLQSGVPSRFSGSGSGTDFTLTISSLQPEDFATYYCQQYNSYP

SEQ ID NO: 284 - protein, 95 aa, Homo sapiens
DIQMTQSPSSLSASVGDRVTITCRASQGIRNDLGWYQQKPGKAPKRLIYAASSLQSGVPSRFSGSGSGTEFTLTISSLQPEDFATYYCLQHNSYP

SEQ ID NO: 285 - protein, 95 aa, Homo sapiens
DIQMTQSPSSLSASVGDRVTITCRASQGISNYLAWYQQKPGKVPKLLIYAASTLQSGVPSRFSGSGSGTDFTLTISSLQPEDVATYYCQKYNSAP

SEQ ID NO: 286 - protein, 95 aa, Homo sapiens
DIQMTQSPSSLSASVGDRVTITCQASQDISNYLNWYQQKPGKAPKLLIYDASNLETGVPSRFSGSGSGTDFTFTISSLQPEDIATYYCQQYDNLP

SEQ ID NO: 287 - protein, 95 aa, Homo sapiens
DIQMTQSPSSLSASVGDRVTITCRASQSISSYLNWYQQKPGKAPKLLIYAASSLQSGVPSRFSGSGSGTDFTLTISSLQPEDFATYYCQQSYSTP

SEQ ID NO: 288 - protein, 95 aa, Homo sapiens
VIWMTQSPSLLSASTGDRVTISCRMSQGISSYLAWYQQKPGKAPELLIYAASTLQSGVPSRFSGSGSGTDFTLTISCLQSEDFATYYCQQYYSFP

SEQ ID NO: 289 - protein, 95 aa, Homo sapiens
AIQLTQSPSSLSASVGDRVTITCRASQGISSALAWYQQKPGKAPKLLIYDASSLESGVPSRFSGSGSGTDFTLTISSLQPEDFATYYCQQFNNYP

SEQ ID NO: 290 - protein, 95 aa, Homo sapiens
DIQMTQSPSSLSASVGDRVTITCRASQGISSWLAWYQQKPEKAPKSLIYAASSLQSGVPSRFSGSGSGTDFTLTISSLQPEDFATYYCQQYNSYP

SEQ ID NO: 291 - protein, 95 aa, Homo sapiens
NIQMTQSPSAMSASVGDRVTITCRARQGISNYLAWFQQKPGKVPKHLIYAASSLQSGVPSRFSGSGSGTEFTLTISSLQPEDFATYYCLQHNSYP

SEQ ID NO: 292 - protein, 95 aa, Homo sapiens
AIRMTQSPFSLSASVGDRVTITCWASQGISSYLAWYQQKPAKAPKLFIYYASSLQSGVPSRFSGSGSGTDYTLTISSLQPEDFATYYCQQYYSTP

SEQ ID NO: 293 - protein, 95 aa, Homo sapiens
DIQMTQSPSSLSASVGDRVTITCRASQGISNSLAWYQQKPGKAPKLLLYAASRLESGVPSRFSGSGSGTDYTLTISSLQPEDFATYYCQQYYSTP

SEQ ID NO: 294 - protein, 100 aa, Homo sapiens
DIVMTQTPLSSPVTLGQPASISCRSSQSLVHSDGNTYLSWLQQRPGQPPRLLIYKISNRFSGVPDRFSGSGAGTDFTLKISRVEAEDVGVYYCMQATQFP

SEQ ID NO: 295 - protein, 100 aa, Homo sapiens
DIVMTQSPLSLPVTPGEPASISCRSSQSLLHSNGYNYLDWYLQKPGQSPQLLIYLGSNRASGVPDRFSGSGSGTDFTLKISRVEAEDVGVYYCMQALQTP

SEQ ID NO: 296 - protein, 100 aa, Homo sapiens
DVVMTQSPLSLPVTLGQPASISCRSSQSLVYSDGNTYLNWFQQRPGQSPRRLIYKVSNRDSGVPDRFSGSGSGTDFTLKISRVEAEDVGVYYCMQGTHWP

SEQ ID NO: 297 - protein, 101 aa, Homo sapiens
DIVMTQTPLSLPVTPGEPASISCRSSQSLLDSDDGNTYLDWYLQKPGQSPQLLIYTLSYRASGVPDRFSGSGSGTDFTLKISRVEAEDVGVYYCMQRIEFP

SEQ ID NO: 298 - protein, 100 aa, Homo sapiens
EIVMTQTPLSLSITPGEQASISCRSSQSLLHSDGYTYLYWFLQKARPVSTLLIYEVSNRFSGVPDRFSGSGSGTDFTLKISRVEAEDFGVYYCMQDAQDP

SEQ ID NO: 299 - protein, 100 aa, Homo sapiens
DIVMTQTPLSLSVTPGQPASISCKSSQSLLHSDGKTYLYWYLQKPGQPPQLLIYEVSNRFSGVPDRFSGSGSGTDFTLKISRVEAEDVGVYYCMQSIQLP

SEQ ID NO: 300 - protein, 100 aa, Homo sapiens
DVVMTQSPLSLPVTLGQPASISCRSSQSLVYSDGNTYLNWFQQRPGQSPRRLIYKVSNWDSGVPDRFSGSGSGTDFTLKISRVEAEDVGVYYCMQGTHWP

SEQ ID NO: 301 - protein, 95 aa, Homo sapiens
EIVLTQSPATLSLSPGERATLSCRASQSVSSYLAWYQQKPGQAPRLLIYDASNRATGIPARFSGSGSGTDFTLTISSLEPEDFAVYYCQQRSNWP

SEQ ID NO: 302 - protein, 95 aa, Homo sapiens
EIVMTQSPATLSVSPGERATLSCRASQSVSSNLAWYQQKPGQAPRLLIYGASTRATGIPARFSGSGSGTEFTLTISSLQSEDFAVYYCQQYNNWP

SEQ ID NO: 303 - protein, 96 aa, Homo sapiens
EIVLTQSPGTLSLSPGERATLSCRASQSVSSSYLAWYQQKPGQAPRLLIYGASSRATGIPDRFSGSGSGTDFTLTISRLEPEDFAVYYCQQYGSSP

SEQ ID NO: 304 - protein, 96 aa, Homo sapiens
EIVMTQSPATLSLSPGERATLSCRASQSVSSSYLSWYQQKPGQAPRLLIYGASTRATGIPARFSGSGSGTDFTLTISSLQPEDFAVYYCQQDYNLP

SEQ ID NO: 305 - protein, 95 aa, Homo sapiens
EIVLTQSPATLSLSPGERATLSCRASQGVSSYLAWYQQKPGQAPRLLIYDASNRATGIPARFSGSGPGTDFTLTISSLEPEDFAVYYCQQRSNWH

SEQ ID NO: 306 - protein, 96 aa, Homo sapiens
EIVLTQSPATLSLSPGERATLSCGASQSVSSSYLAWYQQKPGLAPRLLIYDASSRATGIPDRFSGSGSGTDFTLTISRLEPEDFAVYYCQQYGSSP

SEQ ID NO: 307 - protein, 89 aa, Homo sapiens
EIVLTQSPATLSLSPGERATLSCRASQSVSSYLAWYQQKPGQAPRLLIYGASTRATGIPARFSGSGSGTEFTLTISSLQSEDFAVYYCQ

SEQ ID NO: 308 - protein, 89 aa, Homo sapiens
EIVLTQSPATLSLSPGERATLSCRASQGVSSYLAWYQQKPGQAPRLLIYDASSRATGIPARFSGSGPGTDFTLTISSLEPEDFAVYYCQ

SEQ ID NO: 309 - protein, 90 aa, Homo sapiens
EIVLTQSPGTLSLSPGERATLSCRASQSVSSSYLAWYQQKPGLAPRLLIYGASTRATGIPARFSGSGSGTEFTLTISRLQSEDFAVYYCQ

SEQ ID NO: 310 - protein, 95 aa, Homo sapiens
EIVLTQSPATLSLSPGERATLSCRASQGVSSNLAWYQQKPGQAPRLLIYDASNRATGIPARFSGSGPGTDFTLTISSLEPEDFAVYYCQQRSNWH

SEQ ID NO: 311 - protein, 96 aa, Homo sapiens
EIVLTQSPATLSLSPGERATLSCRASQSVSSSYLAWYQQKPGQAPRLLIYDASSRATGIPDRFSGSGSGTDFTLTISRLEPEDFAVYYCQQRSNWH

SEQ ID NO: 312 - protein, 101 aa, Homo sapiens
DIVMTQSPDSLAVSLGERATINCKSSQSVLYSSNNKNYLAWYQQKPGQPPKLLIYWASTRESGVPDRFSGSGSGTDFTLTISSLQAEDVAVYYCQQYYSTP

SEQ ID NO: 313 - protein, 95 aa, Homo sapiens
ETTLTQSPAFMSATPGDKVNISCKASQDIDDDMNWYQQKPGEAAIFIIQEATTLVPGIPPRFSGSGYGTDFTLTINNIESEDAAYYFCLQHDNFP

SEQ ID NO: 314 - protein, 98 aa, Homo sapiens
QSVLTQPPSVSEAPRQRVTISCSGSSSNIGNNAVNWYQQLPGKAPKLLIYYDDLLPSGVSDRFSGSKSGTSASLAISGLQSEDEADYYCAAWDDSLNG

SEQ ID NO: 315 - protein, 99 aa, Homo sapiens
QSVLTQPPSVSGAPGQRVTISCTGSSSNIGAGYDVHWYQQLPGTAPKLLIYGNSNRPSGVPDRFSGSKSGTSASLAITGLQAEDEADYYCQSYDSSLSG

SEQ ID NO: 316 - protein, 98 aa, Homo sapiens
QSVLTQPPSASGTPGQRVTISCSGSSSNIGSNTVNWYQQLPGTAPKLLIYSNNQRPSGVPDRFSGSKSGTSASLAISGLQSEDEADYYCAAWDDSLNG

SEQ ID NO: 317 - protein, 98 aa, Homo sapiens
QSVLTQPPSASGTPGQRVTISCSGSSSNIGSNYVYWYQQLPGTAPKLLIYRNNQRPSGVPDRFSGSKSGTSASLAISGLRSEDEADYYCAAWDDSLSG

SEQ ID NO: 318 - protein, 98 aa, Homo sapiens
QSVLTQPPSVSAAPGQKVTISCSGSSSNIGNNYVSWYQQLPGTAPKLLIYDNNKRPSGIPDRFSGSKSGTSATLGITGLQTGDEADYYCGTWDSSLSA

SEQ ID NO: 319 - protein, 99 aa, Homo sapiens
QSALTQPPSASGSPGQSVTISCTGTSSDVGGYNYVSWYQQHPGKAPKLMIYEVSKRPSGVPDRFSGSKSGNTASLTVSGLQAEDEADYYCSSYAGSNNF

SEQ ID NO: 320 - protein, 99 aa, Homo sapiens
QSALTQPRSVSGSPGQSVTISCTGTSSDVGGYNYVSWYQQHPGKAPKLMIYDVSKRPSGVPDRFSGSKSGNTASLTISGLQAEDEADYYCCSYAGSYTF

SEQ ID NO: 321 - protein, 99 aa, Homo sapiens
QSALTQPASVSGSPGQSITISCTGTSSDVGGYNYVSWYQQHPGKAPKLMIYEVSNRPSGVSNRFSGSKSGNTASLTISGLQAEDEADYYCSSYTSSSTL

SEQ ID NO: 322 - protein, 99 aa, Homo sapiens
QSALTQPPSVSGSPGQSVTISCTGTSSDVGSYNRVSWYQQPPGTAPKLMIYEVSNRPSGVPDRFSGSKSGNTASLTISGLQAEDEADYYCSLYTSSSTF

SEQ ID NO: 323 - protein, 99 aa, Homo sapiens
QSALTQPASVSGSPGQSITISCTGTSSDVGSYNLVSWYQQHPGKAPKLMIYEGSKRPSGVSNRFSGSKSGNTASLTISGLQAEDEADYYCCSYAGSSTL

SEQ ID NO: 324 - protein, 95 aa, Homo sapiens
SYELTQPPSVSVSPGQTASITCSGDKLGDKYACWYQQKPGQSPVLVIYQDSKRPSGIPERFSGSNSGNTATLTISGTQAMDEADYYCQAWDSSTA

SEQ ID NO: 325 - protein, 95 aa, Homo sapiens
SYELTQPLSVSVALGQTARITCGGNNIGSKNVHWYQQKPGQAPVLVIYRDSNRPSGIPERFSGSNSGNTATLTISRAQAGDEADYYCQVWDSSTA

SEQ ID NO: 326 - protein, 96 aa, Homo sapiens
SYELTQPPSVSVSPGQTARITCSGDALPKKYAYWYQQKSGQAPVLVIYEDSKRPSGIPERFSGSSSGTMATLTISGAQVEDEADYYCYSTDSSGNH

SEQ ID NO: 327 - protein, 96 aa, Homo sapiens
SYELTQPHSVSVATAQMARITCGGNNIGSKAVHWYQQKPGQDPVLVIYSDSNRPSGIPERFSGSNPGNTTTLTISRIEAGDEADYYCQVWDSSSDH

SEQ ID NO: 328 - protein, 96 aa, Homo sapiens
SYELTQPPSVSVSLGQMARITCSGEALPKKYAYWYQQKPGQFPVLVIYKDSERPSGIPERFSGSSSGTIVTLTISGVQAEDEADYYCLSADSSGTY

SEQ ID NO: 329 - protein, 96 aa, Homo sapiens
SSELTQDPAVSVALGQTVRITCQGDSLRSYYASWYQQKPGQAPVLVIYGKNNRPSGIPDRFSGSSSGNTASLTITGAQAEDEADYYCNSRDSSGNH

SEQ ID NO: 330 - protein, 96 aa, Homo sapiens
SYVLTQPPSVSVAPGKTARITCGGNNIGSKSVHWYQQKPGQAPVLVIYYDSDRPSGIPERFSGSNSGNTATLTISRVEAGDEADYYCQVWDSSSDH

SEQ ID NO: 331 - protein, 94 aa, Homo sapiens
SYELTQLPSVSVSPGQTARITCSGDVLGENYADWYQQKPGQAPELVIYEDSERYPGIPERFSGSTSGNTTTLTISRVLTEDEADYYCLSGDEDN

SEQ ID NO: 332 - protein, 96 aa, Homo sapiens
SYELMQPPSVSVSPGQTARITCSGDALPKQYAYWYQQKPGQAPVLVIYKDSERPSGIPERFSGSSSGTTVTLTISGVQAEDEADYYCQSADSSGTY

SEQ ID NO: 333 - protein, 94 aa, Homo sapiens
SYELTQPSSVSVSPGQTARITCSGDVLAKKYARWFQQKPGQAPVLVIYKDSERPSGIPERFSGSSSGTTVTLTISGAQVEDEADYYCYSAADNN

SEQ ID NO: 334 - protein, 103 aa, Homo sapiens
LPVLTQPPSASALLGASIKLTCTLSSEHSTYTIEWYQQRPGRSPQYIMKVKSDGSHSKGDGIPDRFMGSSSGADRYLTFSNLQSDDEAEYHCGESHTIDGQVG

SEQ ID NO: 335 - protein, 99 aa, Homo sapiens
QPVLTQSSSASASLGSSVKLTCTLSSGHSSYIIAWHQQQPGKAPRYLMKLEGSGSYNKGSGVPDRFSGSSSGADRYLTISNLQLEDEADYYCETWDSNT

SEQ ID NO: 336 - protein, 99 aa, Homo sapiens
QLVLTQSPSASASLGASVKLTCTLSSGHSSYAIAWHQQQPEKGPRYLMKLNSDGSHSKGDGIPDRFSGSSSGAERYLTISSLQSEDEADYYCQTWGTGI

SEQ ID NO: 337 - protein, 104 aa, Homo sapiens
QPVLTQPPSSSASPGESARLTCTLPSDINVGSYNIYWYQQKPGSPPRYLLYYYSDSDKGQGSGVPSRFSGSKDASANTGILLISGLQSEDEADYYCMIWPSNAS

SEQ ID NO: 338 - protein, 104 aa, Homo sapiens
QPVLTQPTSLSASPGASARFTCTLRSGINVGTYRIYWYQQKPGSLPRYLLRYKSDSDKQQGSGVPSRFSGSKDASTNAGLLLISGLQSEDEADYYCAIWYSSTS

SEQ ID NO: 339 - protein, 104 aa, Homo sapiens
QAVLTQPASLSASPGASASLTCTLRSGINVGTYRIYWYQQKPGSPPQYLLRYKSDSDKQQGSGVPSRFSGSKDASANAGILLISGLQSEDEADYYCMIWHSSAS

SEQ ID NO: 340 - protein, 105 aa, Homo sapiens
QPVLTQPSSHSASSGASVRLTCMLSSGFSVGDFWIRWYQQKPGNPPRYLLYYHSDSNKGQGSGVPSRFSGSNDASANAGILRISGLQPEDEADYYCGTWHSNSKT

SEQ ID NO: 341 - protein, 98 aa, Homo sapiens
NFMLTQPHSVSESPGKTVTISCTRSSGSIASNYVQWYQQRPGSSPTTVIYEDNQRPSGVPDRFSGSIDSSSNSASLTISGLKTEDEADYYCQSYDSSN

SEQ ID NO: 342 - protein, 98 aa, Homo sapiens
QTVVTQEPSLTVSPGGTVTLTCASSTGAVTSGYYPNWFQQKPGQAPRALIYSTSNKHSWTPARFSGSLLGGKAALTLSGVQPEDEAEYYCLLYYGGAQ

SEQ ID NO: 343 - protein, 98 aa, Homo sapiens
QAVVTQEPSLTVSPGGTVTLTCGSSTGAVTSGHYPYWFQQKPGQAPRTLIYDTSNKHSWTPARFSGSLLGGKAALTLSGAQPEDEAEYYCLLSYSGAR

SEQ ID NO: 344 - protein, 98 aa, Homo sapiens
QTVVTQEPSFSVSPGGTVTLTCGLSSGSVSTSYYPSWYQQTPGQAPRTLIYSTNTRSSGVPDRFSGSILGNKAALTITGAQADDESDYYCVLYMGSGI

SEQ ID NO: 345 - protein, 104 aa, Homo sapiens
QPVLTQPPSASASLGASVTLTCTLSSGYSNYKVDWYQQRPGKGPRFVMRVGTGGIVGSKGDGIPDRFSVLGSGLNRYLTIKNIQEEDESDYHCGADHGSGSNFV

SEQ ID NO: 346 - protein, 98 aa, Homo sapiens
QAGLTQPPSVSKGLRQTATLTCTGNSNNVGNQGAAWLQQHQGHPPKLLSYRNNNRPSGISERLSASRSGNTASLTITGLQPEDEADYYCSAWDSSLSA

SEQ ID NO: 347 - protein, 98 aa, Homo sapiens
QVQLVQSGAEVKKPGASVKVSCKASGYTFTGYYMHWVRQAPGQGLEWMGRINPNSGGTNYAQKFQGRVTSTRDTSISTAYMELSRLRSDDTVVYYCAR

SEQ ID NO: 348 - protein, 98 aa, Homo sapiens
QVQLVQSGAEVKKPGASVKVSCKASGYTFTSYAMHWVRQAPGQRLEWMGWINAGNGNTKYSQKFQGRVTITRDTSASTAYMELSSLRSEDTAVYYCAR

SEQ ID NO: 349 - protein, 98 aa, Homo sapiens
QVQLVQSGAEVKKPGASVKVSCKASGYTFTSYDINWVRQATGQGLEWMGWMNPNSGNTGYAQKFQGRVTMTRNTSISTAYMELSSLRSEDTAVYYCAR

SEQ ID NO: 350 - protein, 98 aa, Homo sapiens
QVQLVQSGAEVKKPGASVKVSCKASGYTFTSYGISWVRQAPGQGLEWMGWISAYNGNTNYAQKLQGRVTMTTDTSTSTAYMELRSLRSDDTAVYYCAR

SEQ ID NO: 351 - protein, 98 aa, Homo sapiens
QVQLVQSGAEVKKPGASVKVSCKVSGYTLTELSMHWVRQAPGKGLEWMGGFDPEDGETIYAQKFQGRVTMTEDTSTDTAYMELSSLRSEDTAVYYCAT

SEQ ID NO: 352 - protein, 98 aa, Homo sapiens
QMQLVQSGAEVKKTGSSVKVSCKASGYTFTYRYLHWVRQAPGQALEWMGWITPFNGNTNYAQKFQDRVTITRDRSMSTAYMELSSLRSEDTAMYYCAR

SEQ ID NO: 353 - protein, 98 aa, Homo sapiens
QVQLVQSGAEVKKPGASVKVSCKASGYTFTSYYMHWVRQAPGQGLEWMGIINPSGGSTSYAQKFQGRVTMTRDTSTSTVYMELSSLRSEDTAVYYCAR

SEQ ID NO: 354 - protein, 98 aa, Homo sapiens
QMQLVQSGPEVKKPGTSVKVSCKASGFTFTSSAVQWVRQARGQRLEWIGWIVVGSGNTNYAQKFQERVTITRDMSTSTAYMELSSLRSEDTAVYYCAA

SEQ ID NO: 355 - protein, 98 aa, Homo sapiens
EVQLVQSGAEVKKPGATVKISCKVSGYTFTDYYMHWVQQAPGKGLEWMGLVDPEDGETIYAEKFQGRVTITADTSTDTAYMELSSLRSEDTAVYYCAT

SEQ ID NO: 356 - protein, 98 aa, Homo sapiens
QVQLVQSGAEVKKPGSSVKVSCKASGGTFSSYAISWVRQAPGQGLEWMGGIIPIFGTANYAQKFQGRVTITADESTSTAYMELSSLRSEDTAVYYCAR

SEQ ID NO: 357 - protein, 100 aa, Homo sapiens
QITLKESGPTLVKPTQTLTLTCTFSGFSLSTSGVGVGWIRQPPGKALEWLALIYWNDDKRYSPSLKSRLTITKDTSKNQVVLTMTNMDPVDTATYYCAHR

SEQ ID NO: 358 - protein, 100 aa, Homo sapiens
QVTLKESGPVLVKPTETLTLTCTVSGFSLSNARMGVSWIRQPPGKALEWLAHIFSNDEKSYSTSLKSRLTISKDTSKSQVVLTMTNMDPVDTATYYCARI

SEQ ID NO: 359 - protein, 100 aa, Homo sapiens
QVTLRESGPALVKPTQTLTLTCTFSGFSLSTSGMCVSWIRQPPGKALEWLALIDWDDDKYYSTSLKTRLTISKDTSKNQVVLTMTNMDPVDTATYYCARI

SEQ ID NO: 360 - protein, 98 aa, Homo sapiens
EVQLVESGGGLVQPGGSLRLSCAASGFTFSSYWMSWVRQAPGKGLEWVANIKQDGSEKYYVDSVKGRFTISRDNAKNSLYLQMNSLRAEDTAVYYCAR

SEQ ID NO: 361 - protein, 99 aa, Homo sapiens
EVQLVESGGGLVQPGRSLRLSCAASGFTFDDYAMHWVRQAPGKGLEWVSGISWNSGSIGYADSVKGRFTISRDNAKNSLYLQMNSLRAEDTALYYCAKD

SEQ ID NO: 362 - protein, 98 aa, Homo sapiens
QVQLVESGGGLVKPGGSLRLSCAASGFTFSDYYMSWIRQAPGKGLEWVSYISSSGSTIYYADSVKGRFTISRDNAKNSLYLQMNSLRAEDTAVYYCAR

SEQ ID NO: 363 - protein, 97 aa, Homo sapiens
EVQLVESGGGLVQPGGSLRLSCAASGFTFSSYDMHWVRQATGKGLEWVSAIGTAGDTYYPGSVKGRFTISRENAKNSLYLQMNSLRAGDTAVYYCAR

SEQ ID NO: 364 - protein, 100 aa, Homo sapiens
EVQLVESGGGLVKPGGSLRLSCAASGFTFSNAWMSWVRQAPGKGLEWVGRIKSKTDGGTTDYAAPVKGRFTISRDDSKNTLYLQMNSLKTEDTAVYYCTT

SEQ ID NO: 365 - protein, 98 aa, Homo sapiens
EVQLVESGGGVVRPGGSLRLSCAASGFTFDDYGMSWVRQAPGKGLEWVSGINWNGGSTGYADSVKGRFTISRDNAKNSLYLQMNSLRAEDTALYHCAR

SEQ ID NO: 366 - protein, 98 aa, Homo sapiens
EVQLVESGGGLVKPGGSLRLSCAASGFTFSSYSMNWVRQAPGKGLEWVSSISSSSSYIYYADSVKGRFTISRDNAKNSLYLQMNSLRAEDTAVYYCAR

SEQ ID NO: 367 - protein, 98 aa, Homo sapiens
EVQLLESGGGLVQPGGSLRLSCAASGFTFSSYAMSWVRQAPGKGLEWVSAISGSGGSTYYADSVKGRFTISRDNSKNTLYLQMNSLRAEDTAVYYCAK

SEQ ID NO: 368 - protein, 98 aa, Homo sapiens
QVQLVESGGGVVQPGRSLRLSCAASGFTFSSYAMHWVRQAPGKGLEWVAVISYDGSNKYYADSVKGRFTISRDNSKNTLYLQMNSLRAEDTAVYYCAR

SEQ ID NO: 369 - protein, 98 aa, Homo sapiens
QVQLVESGGGVVQPGRSLRLSCAASGFTFSSYGMHWVRQAPGKGLEWVAVIWYDGSNKYYADSVKGRFTISRDNSKNTLYLQMNSLRAEDTAVYYCAR

SEQ ID NO: 370 - protein, 99 aa, Homo sapiens
EVQLVESGGVVVQPGGSLRLSCAASGFTFDDYTMHWVRQAPGKGLEWVSLISWDGGSTYYADSVKGRFTISRDNSKNSLYLQMNSLRTEDTALYYCAKD

SEQ ID NO: 371 - protein, 98 aa, Homo sapiens
EVQLVESGGGLVQPGGSLRLSCAASGFTFSSYSMNWVRQAPGKGLEWVSYISSSSSTIYYADSVKGRFTISRDNAKNSLYLQMNSLRAEDTAVYYCAR

SEQ ID NO: 372 - protein, 100 aa, Homo sapiens
EVQLVESGGGLVQPGRSLRLSCTASGFTFGDYAMSWFRQAPGKGLEWVGFIRSKAYGGTTEYTASVKGRFTISRDGSKSIAYLQMNSLKTEDTAVYYCTR

SEQ ID NO: 373 - protein, 97 aa, Homo sapiens
EVQLVESGGGLIQPGGSLRLSCAASGFTVSSNYMSWVRQAPGKGLEWVSVIYSGGSTYYADSVKGRFTISRDNSKNTLYLQMNSLRAEDTAVYYCAR

SEQ ID NO: 374 - protein, 98 aa, Homo sapiens
EVQLVESGGGLVQPGGSLRLSCAASGFTFSSYAMHWVRQAPGKGLEYVSAISSNGGSTYYANSVKGRFTISRDNSKNTLYLQMGSLRAEDMAVYYCAR

SEQ ID NO: 375 - protein, 97 aa, Homo sapiens
EVQLVESGGGLVQPGGSLRLSCAASGFTVSSNYMSWVRQAPGKGLEWVSVIYSGGSTYYADSVKGRFTISRDNSKNTLYLQMNSLRAEDTAVYYCAR

SEQ ID NO: 376 - protein, 100 aa, Homo sapiens
EVQLVESGGGLVQPGGSLRLSCAASGFTFSDHYMDWVRQAPGKGLEWVGRTRNKANSYTTEYAASVKGRFTISRDDSKNSLYLQMNSLKTEDTAVYYCAR

SEQ ID NO: 377 - protein, 100 aa, Homo sapiens
EVQLVESGGGLVQPGGSLKLSCAASGFTFSGSAMHWVRQASGKGLEWVGRIRSKANSYATAYAASVKGRFTISRDDSKNTAYLQMNSLKTEDTAVYYCTR

SEQ ID NO: 378 - protein, 98 aa, Homo sapiens
EVQLVESGGGLVQPGGSLRLSCAASGFTFSSYWMHWVRQAPGKGLVWVSRINSDGSSTSYADSVKGRFTISRDNAKNTLYLQMNSLRAEDTAVYYCAR

SEQ ID NO: 379 - protein, 96 aa, Homo sapiens
EVQLVESRGVLVQPGGSLRLSCAASGFTVSSNEMSWVRQAPGKGLEWVSSISGGSTYYADSRKGRFTISRDNSKNTLHLQMNSLRAEDTAVYYCKK

SEQ ID NO: 380 - protein, 98 aa, Homo sapiens
QVQLVESGGGVVQPGGSLRLSCAASGFTFSSYGMHWVRQAPGKGLEWVSVIYSGGSSTYYADSVKGRFTISRDNSKNTLYLQMNSLRAEDTAVYYCAK

SEQ ID NO: 381 - protein, 98 aa, Homo sapiens
QVQLQESGPGLVKPPGTLSLTCAVSGGSISSSNWWSWVRQPPGKGLEWIGEIYHSGSTNYNPSLKSRVTISVDKSKNQFSLKLSSVTAADTAVYCCAR

SEQ ID NO: 382 - protein, 98 aa, Homo sapiens
QVQLQESGPGLVKPSDTLSLTCAVSGYSISSSNWWGWIRQPPGKGLEWIGYIYYSGSTYYNPSLKSRVTMSVDTSKNQFSLKLSSVTAVDTAVYYCAR

SEQ ID NO: 383 - protein, 99 aa, Homo sapiens
QLQLQESGSGLVKPSQTLSLTCAVSGGSISSGGYSWSWIRQPPGKGLEWIGYIYHSGSTYYNPSLKSRVTISVDRSKNQFSLKLSSVTAADTAVYYCAR

SEQ ID NO: 384 - protein, 99 aa, Homo sapiens
QVQLQESGPGLVKPSQTLSLTCTVSGGSISSGDYYWSWIRQPPGKGLEWIGYIYYSGSTYYNPSLKSRVTISVDTSKNQFSLKLSSVTAADTAVYYCAR

SEQ ID NO: 385 - protein, 99 aa, Homo sapiens
QVQLQESGPGLVKPSQTLSLTCTVSGGSISSGGYYWSWIRQHPGKGLEWIGYIYYSGSTYYNPSLKSLVTISVDTSKNQFSLKLSSVTAADTAVYYCAR

SEQ ID NO: 386 - protein, 97 aa, Homo sapiens
QVQLQQWGAGLLKPSETLSLTCAVYGGSFSGYYWSWIRQPPGKGLEWIGEINHSGSTNYNPSLKSRVTISVDTSKNQFSLKLSSVTAADTAVYYCAR

SEQ ID NO: 387 - protein, 99 aa, Homo sapiens
QLQLQESGPGLVKPSETLSLTCTVSGGSISSSSYYWGWIRQPPGKGLEWIGSIYYSGSTYYNPSLKSRVTISVDTSKNQFSLKLSSVTAADTAVYYCAR

SEQ ID NO: 388 - protein, 97 aa, Homo sapiens
QVQLQESGPGLVKPSETLSLTCTVSGGSISSYYWSWIRQPPGKGLEWIGYIYYSGSTNYNPSLKSRVTISVDTSKNQFSLKLSSVTAADTAVYYCAR

SEQ ID NO: 389 - protein, 98 aa, Homo sapiens
QVQLQESGPGLVKPSETLSLTCAVSGYSISSGYYWGWIRQPPGKGLEWIGSIYHSGSTYYNPSLKSRVTISVDTSKNQFSLKLSSVTAADTAVYYCAR

SEQ ID NO: 390 - protein, 99 aa, Homo sapiens
QVQLQESGPGLVKPSETLSLTCTVSGGSVSSGSYYWSWIRQPPGKGLEWIGYIYYSGSTNYNPSLKSRVTISVDTSKNQFSLKLSSVTAADTAVYYCAR

SEQ ID NO: 391 - protein, 98 aa, Homo sapiens
EVQLVQSGAEVKKPGESLRISCKGSGYSFTSYWISWVRQMPGKGLEWMGRIDPSDSYTNYSPSFQGHVTISADKSISTAYLQWSSLKASDTAMYYCAR

SEQ ID NO: 392 - protein, 98 aa, Homo sapiens
EVQLVQSGAEVKKPGESLKISCKGSGYSFTSYWIGWVRQMPGKGLEWMGIIYPGDSDTRYSPSFQGQVTISADKSISTAYLQWSSLKASDTAMYYCAR

SEQ ID NO: 393 - protein, 101 aa, Homo sapiens
QVQLQQSGPGLVKPSQTLSLTCAISGDSVSSNSAAWNWIRQSPSRGLEWLGRTYYRSKWYNDYAVSVKSRITINPDTSKNQFSLQLNSVTPEDTAVYYCAR

SEQ ID NO: 394 - protein, 98 aa, Homo sapiens
QVQLVQSGSELKKPGASVKVSCKASGYTFTSYAMNWVRQAPGQGLEWMGWINTNTGNPTYAQGFTGRFVFSLDTSVSTAYLQICSLKAEDTAVYYCAR

SEQ ID NO: 395 - protein, 12 aa, Homo sapiens
WTFGQGTKVEIK

SEQ ID NO: 396 - protein, 12 aa, Homo sapiens
YTFGQGTKLEIK

SEQ ID NO: 397 - protein, 12 aa, Homo sapiens
FTFGPGTKVDIK

SEQ ID NO: 398 - protein, 12 aa, Homo sapiens
LTFGGGTKVEIK

SEQ ID NO: 399 - protein, 12 aa, Homo sapiens
ITFGQGTRLEIK

SEQ ID NO: 400 - protein, 12 aa, Homo sapiens
YVFGTGTKVTVL

SEQ ID NO: 401 - protein, 12 aa, Homo sapiens
VVFGGGTKLTVL

SEQ ID NO: 402 - protein, 12 aa, Homo sapiens
NVFGSGTKVTVL

SEQ ID NO: 403 - protein, 12 aa, Homo sapiens
AVFGGGTQLTVL

SEQ ID NO: 404 - protein, 17 aa, Homo sapiens
AEYFQHWGQGTLVTVSS

SEQ ID NO: 405 - protein, 17 aa, Homo sapiens
YWYFDLWGRGTLVTVSS

SEQ ID NO: 406 - protein, 16 aa, Homo sapiens
DAFDVWGQGTMVTVSS

SEQ ID NO: 407 - protein, 15 aa, Homo sapiens
YFDYWGQGTLVTVSS

SEQ ID NO: 408 - protein, 16 aa, Homo sapiens
NWFDSWGQGTLVTVSS

SEQ ID NO: 409 - protein, 20 aa, Homo sapiens
YYYYYGMDVWGQGTTVTVSS

SEQ ID NO: 410 - protein, 20 aa, Homo sapiens
VQKYTRALHDSSITGISPIT

SEQ ID NO: 411 - protein, 20 aa, Homo sapiens
SSITGISPITEYLASLSTYN

SEQ ID NO: 412 - protein, 20 aa, Homo sapiens
EYLASLSTYNDQSITFALED

SEQ ID NO: 413 - protein, 20 aa, Homo sapiens
DQSITFALEDESYEIYVEDL

SEQ ID NO: 414 - protein, 20 aa, Homo sapiens
ESYEIYVEDLKKDEKKDKVL

SEQ ID NO: 415 - protein, 20 aa, Homo sapiens
KKDEKKDKVLLSYYESQHPS

SEQ ID NO: 416 - protein, 20 aa, Homo sapiens
LSYYESQHPSNESGDGVDGK

SEQ ID NO: 417 - protein, 20 aa, Homo sapiens
NESGDGVDGKMLMVTLSPTK

SEQ ID NO: 418 - protein, 20 aa, Homo sapiens
MLMVTLSPTKDFWLHANNKE

SEQ ID NO: 419 - protein, 20 aa, Homo sapiens
DFWLHANNKEHSVELHKCEK

SEQ ID NO: 420 - protein, 20 aa, Homo sapiens
HSVELHKCEKPLPDQAFFVL

SEQ ID NO: 421 - protein, 20 aa, Homo sapiens
PLPDQAFFVLHNMHSNCVSF

SEQ ID NO: 422 - protein, 20 aa, Homo sapiens
HNMHSNCVSFECKTDPGVFI

SEQ ID NO: 423 - protein, 20 aa, Homo sapiens
ECKTDPGVFIGVKDNHLALI

SEQ ID NO: 424 - protein, 20 aa, Homo sapiens
GVKDNHLALIKVDSSENLCT

SEQ ID NO: 425 - protein, 20 aa, Homo sapiens
KVDSSENLCTENILFKLSET

SEQ ID NO: 426 - protein, 10 aa, Homo sapiens
LEDESYEIYV

SEQ ID NO: 427 - protein, 9 aa, Homo sapiens
EDESYEIYV